European Patent Specification EP 4 146 683 B1, published January 28, 2026. Title: APRIL AND BAFF INHIBITORY IMMUNOMODULATORY PROTEINS AND METHODS OF USE THEREOF. Applicant: ALPINE IMMUNE SCIENCES, INC. Application Not Yet Assigned. The sequence listing filed with the application follows.

SEQUENCE LISTING (239 sequences)

SEQ ID NO: 1 - protein, 82 aa, ARTIFICIAL SEQUENCE
  TACI WT ECD
VAMRSCPEEQYWDPLLGTCMSCKTICNHQSQRTCAAFCRSLSCRKEQGKFYDHLLRDCISCASICGQHPKQCAYFCENKLRS

SEQ ID NO: 2 - protein, 82 aa, ARTIFICIAL SEQUENCE
  TACI L82P ECD
VAMRSCPEEQYWDPLLGTCMSCKTICNHQSQRTCAAFCRSLSCRKEQGKFYDHPLRDCISCASICGQHPKQCAYFCENKLRS

SEQ ID NO: 3 - protein, 82 aa, ARTIFICIAL SEQUENCE
  TACI D85E, K98T ECD
VAMRSCPEEQYWDPLLGTCMSCKTICNHQSQRTCAAFCRSLSCRKEQGKFYDHLLRECISCASICGQHPTQCAYFCENKLRS

SEQ ID NO: 4 - protein, 82 aa, ARTIFICIAL SEQUENCE
  TACI I87L, K98T ECD
VAMRSCPEEQYWDPLLGTCMSCKTICNHQSQRTCAAFCRSLSCRKEQGKFYDHLLRDCLSCASICGQHPTQCAYFCENKLRS

SEQ ID NO: 5 - protein, 82 aa, ARTIFICIAL SEQUENCE
  TACI R60G, Q75E, L82P ECD
VAMRSCPEEQYWDPLLGTCMSCKTICNHQSQGTCAAFCRSLSCRKEEGKFYDHPLRDCISCASICGQHPKQCAYFCENKLRS

SEQ ID NO: 6 - protein, 82 aa, ARTIFICIAL SEQUENCE
  TACI R60G, C86Y ECD
VAMRSCPEEQYWDPLLGTCMSCKTICNHQSQGTCAAFCRSLSCRKEQGKFYDHLLRDYISCASICGQHPKQCAYFCENKLRS

SEQ ID NO: 7 - protein, 82 aa, ARTIFICIAL SEQUENCE
  TACI A101D ECD
VAMRSCPEEQYWDPLLGTCMSCKTICNHQSQRTCAAFCRSLSCRKEQGKFYDHLLRDCISCASICGQHPKQCDYFCENKLRS

SEQ ID NO: 8 - protein, 82 aa, ARTIFICIAL SEQUENCE
  TACI C86Y ECD
VAMRSCPEEQYWDPLLGTCMSCKTICNHQSQRTCAAFCRSLSCRKEQGKFYDHLLRDYISCASICGQHPKQCAYFCENKLRS

SEQ ID NO: 9 - protein, 82 aa, ARTIFICIAL SEQUENCE
  TACI W40R, L82P, F103Y ECD
VAMRSCPEEQYRDPLLGTCMSCKTICNHQSQRTCAAFCRSLSCRKEQGKFYDHPLRDCISCASICGQHPKQCAYYCENKLRS

SEQ ID NO: 10 - protein, 82 aa, ARTIFICIAL SEQUENCE
  TACI W40R, Q59R, T61P, K98T ECD
VAMRSCPEEQYRDPLLGTCMSCKTICNHQSRRPCAAFCRSLSCRKEQGKFYDHLLRDCISCASICGQHPTQCAYFCENKLRS

SEQ ID NO: 11 - protein, 82 aa, ARTIFICIAL SEQUENCE
  TACI L82P, I87L ECD
VAMRSCPEEQYWDPLLGTCMSCKTICNHQSQRTCAAFCRSLSCRKEQGKFYDHPLRDCLSCASICGQHPKQCAYFCENKLRS

SEQ ID NO: 12 - protein, 82 aa, ARTIFICIAL SEQUENCE
  TACI G76S, P97S ECD
VAMRSCPEEQYWDPLLGTCMSCKTICNHQSQRTCAAFCRSLSCRKEQSKFYDHLLRDCISCASICGQHSKQCAYFCENKLRS

SEQ ID NO: 13 - protein, 43 aa, ARTIFICIAL SEQUENCE
  TACI WT ECD
SLSCRKEQGKFYDHLLRDCISCASICGQHPKQCAYFCENKLRS

SEQ ID NO: 14 - protein, 43 aa, ARTIFICIAL SEQUENCE
  TACI D85V ECD
SLSCRKEQGKFYDHLLRVCISCASICGQHPKQCAYFCENKLRS

SEQ ID NO: 15 - protein, 43 aa, ARTIFICIAL SEQUENCE
  TACI E74V ECD
SLSCRKVQGKFYDHLLRDCISCASICGQHPKQCAYFCENKLRS

SEQ ID NO: 16 - protein, 43 aa, ARTIFICIAL SEQUENCE
  TACI R84L ECD
SLSCRKEQGKFYDHLLLDCISCASICGQHPKQCAYFCENKLRS

SEQ ID NO: 17 - protein, 43 aa, ARTIFICIAL SEQUENCE
  TACI K77E, R84L, F103Y ECD
SLSCRKEQGEFYDHLLLDCISCASICGQHPKQCAYYCENKLRS

SEQ ID NO: 18 - protein, 43 aa, ARTIFICIAL SEQUENCE
  TACI Y79F, Q99E ECD
SLSCRKEQGKFFDHLLRDCISCASICGQHPKECAYFCENKLRS

SEQ ID NO: 19 - protein, 43 aa, ARTIFICIAL SEQUENCE
  TACI Y79F ECD
SLSCRKEQGKFFDHLLRDCISCASICGQHPKQCAYFCENKLRS

SEQ ID NO: 20 - protein, 43 aa, ARTIFICIAL SEQUENCE
  TACI R84G ECD
SLSCRKEQGKFYDHLLGDCISCASICGQHPKQCAYFCENKLRS

SEQ ID NO: 21 - protein, 82 aa, ARTIFICIAL SEQUENCE
  TACI L83S, F103S ECD
VAMRSCPEEQYWDPLLGTCMSCKTICNHQSQRTCAAFCRSLSCRKEQGKFYDHLSRDCISCASICGQHPKQCAYSCENKLRS

SEQ ID NO: 22 - protein, 82 aa, ARTIFICIAL SEQUENCE
  TACI L82H ECD
VAMRSCPEEQYWDPLLGTCMSCKTICNHQSQRTCAAFCRSLSCRKEQGKFYDHHLRDCISCASICGQHPKQCAYFCENKLRS

SEQ ID NO: 23 - protein, 43 aa, ARTIFICIAL SEQUENCE
  TACI A101D ECD
SLSCRKEQGKFYDHLLRDCISCASICGQHPKQCDYFCENKLRS

SEQ ID NO: 24 - protein, 43 aa, ARTIFICIAL SEQUENCE
  TACI K77E, R84Q ECD
SLSCRKEQGEFYDHLLQDCISCASICGQHPKQCAYFCENKLRS

SEQ ID NO: 25 - protein, 43 aa, ARTIFICIAL SEQUENCE
  TACI K77E, A101D ECD
SLSCRKEQGEFYDHLLRDCISCASICGQHPKQCDYFCENKLRS

SEQ ID NO: 26 - protein, 43 aa, ARTIFICIAL SEQUENCE
  TACI K77E, F78Y, Y102D ECD
SLSCRKEQGEYYDHLLRDCISCASICGQHPKQCADFCENKLRS

SEQ ID NO: 27 - protein, 43 aa, ARTIFICIAL SEQUENCE
  TACI Q75E, R84Q ECD
SLSCRKEEGKFYDHLLQDCISCASICGQHPKQCAYFCENKLRS

SEQ ID NO: 28 - protein, 43 aa, ARTIFICIAL SEQUENCE
  TACI Q75R, R84G, I92V ECD
SLSCRKERGKFYDHLLGDCISCASVCGQHPKQCAYFCENKLRS

SEQ ID NO: 29 - protein, 43 aa, ARTIFICIAL SEQUENCE
  TACI K77E, A101D, Y102D ECD
SLSCRKEQGEFYDHLLRDCISCASICGQHPKQCDDFCENKLRS

SEQ ID NO: 30 - protein, 43 aa, ARTIFICIAL SEQUENCE
  TACI R84Q ECD
SLSCRKEQGKFYDHLLQDCISCASICGQHPKQCAYFCENKLRS

SEQ ID NO: 31 - protein, 43 aa, ARTIFICIAL SEQUENCE
  TACI R84Q, S88N, A101D ECD
SLSCRKEQGKFYDHLLQDCINCASICGQHPKQCDYFCENKLRS

SEQ ID NO: 32 - protein, 43 aa, ARTIFICIAL SEQUENCE
  TACI K77E ECD
SLSCRKEQGEFYDHLLRDCISCASICGQHPKQCAYFCENKLRS

SEQ ID NO: 33 - protein, 43 aa, ARTIFICIAL SEQUENCE
  TACI R84Q, F103V ECD
SLSCRKEQGKFYDHLLQDCISCASICGQHPKQCAYVCENKLRS

SEQ ID NO: 34 - protein, 43 aa, ARTIFICIAL SEQUENCE
  TACI K77E, Q95R, A101D ECD
SLSCRKEQGEFYDHLLRDCISCASICGRHPKQCDYFCENKLRS

SEQ ID NO: 35 - protein, 43 aa, ARTIFICIAL SEQUENCE
  TACI I87M, A101D ECD
SLSCRKEQGKFYDHLLRDCMSCASICGQHPKQCDYFCENKLRS

SEQ ID NO: 36 - DNA, 246 bp, ARTIFICIAL SEQUENCE
  TACI WT ECD
gtggcaatgcgctcatgcccagaggaacaatattgggatccgcttcttgggacgtgtatgagctgcaagaccatctgtaatcatcaatcccaaaggacatgcgcagctttctgcaggagtctctcttgcaggaaagagcaaggcaaattttacgaccatcttttgcgagactgtataagctgtgcgtctatttgtggacaacaccctaaacaatgtgcttatttctgtgaaaataagcttcgatct

SEQ ID NO: 37 - DNA, 246 bp, ARTIFICIAL SEQUENCE
  TACI L82P ECD
gtggcaatgcgctcatgcccagaggaacaatattgggatccgcttcttgggacgtgtatgagctgcaagaccatctgtaatcatcaatcccaaaggacatgcgcagctttctgcaggagtctctcttgcaggaaagagcaaggcaaattttacgaccatcctttgcgagactgtataagctgtgcgtctatttgtggacaacaccctaaacaatgtgcttatttctgtgaaaataagcttcgatct

SEQ ID NO: 38 - DNA, 246 bp, ARTIFICIAL SEQUENCE
  TACI D85E, K98T ECD
gtggcaatgcgctcatgcccagaggaacaatattgggatccgcttcttgggacgtgtatgagctgcaagaccatctgtaatcatcaatcccaaaggacatgcgcagctttctgcaggagtctctcttgcaggaaagagcaaggcaaattttacgaccatcttttgcgagaatgtataagctgtgcgtctatttgtggacaacaccctacacaatgtgcttatttctgtgaaaataagcttcgatct

SEQ ID NO: 39 - DNA, 246 bp, ARTIFICIAL SEQUENCE
  TACI I87L, K98T ECD
gtggcaatgcgctcatgcccagaggaacaatattgggatccgcttcttgggacgtgtatgagctgcaagaccatctgtaatcatcaatcccaaaggacatgcgcagctttctgcaggagtctctcttgcaggaaagagcaaggcaaattttacgaccatcttttgcgagactgtttaagctgtgcgtctatttgtggacaacaccctacacaatgtgcttatttctgtgaaaataagcttcgatct

SEQ ID NO: 40 - DNA, 246 bp, ARTIFICIAL SEQUENCE
  TACI R60G, Q75E, L82P ECD
gtggcaatgcgctcatgcccagaggaacaatattgggatccgcttcttgggacgtgtatgagctgcaagaccatctgtaatcatcaatcccaagggacatgcgcagctttctgcaggagtctctcttgcaggaaagaggaaggcaaattttacgaccatcctttgcgagactgtataagctgtgcgtctatttgtggacaacaccctaaacaatgtgcttatttctgtgaaaataagcttcgatct

SEQ ID NO: 41 - DNA, 246 bp, ARTIFICIAL SEQUENCE
  TACI R60G, C86Y ECD
gtggcaatgcgctcatgcccagaggaacaatattgggatccgcttcttgggacgtgtatgagctgcaagaccatctgtaatcatcaatcccaagggacatgcgcagctttctgcaggagtctctcttgcaggaaagagcaaggcaaattttacgaccatcttttgcgagactacataagctgtgcgtctatttgtggacaacaccctaaacaatgtgcttatttctgtgaaaataagcttcgatct

SEQ ID NO: 42 - DNA, 246 bp, ARTIFICIAL SEQUENCE
  TACI A101D ECD
gtggcaatgcgctcatgcccagaggaacaatattgggatccgcttcttgggacgtgtatgagctgcaagaccatctgtaatcatcaatcccaaaggacatgcgcagctttctgcaggagtctctcttgcaggaaagagcaaggcaaattttacgaccatcttttgcgagactgtataagctgtgcgtctatttgtggacaacaccctaaacaatgtgattatttctgtgaaaataagcttcgatct

SEQ ID NO: 43 - DNA, 246 bp, ARTIFICIAL SEQUENCE
  TACI C86Y ECD
gtggcaatgcgctcatgcccagaggaacaatattgggatccgcttcttgggacgtgtatgagctgcaagaccatctgtaatcatcaatcccaaaggacatgcgcagctttctgcaggagtctctcttgcaggaaagagcaaggcaaattttacgaccatcttttgcgagactatataagctgtgcgtctatttgtggacaacaccctaaacaatgtgcttatttctgtgaaaataagcttcgatct

SEQ ID NO: 44 - DNA, 246 bp, ARTIFICIAL SEQUENCE
  TACI W40R, L82P, F103Y ECD
gtggcaatgcgctcatgcccagaggaacaatatcgggatccgcttcttgggacgtgtatgagctgcaagaccatctgtaatcatcaatcccaaaggacatgcgcagctttctgcaggagtctctcttgcaggaaagagcaaggcaaattttacgaccatcctttgcgagactgtataagctgtgcgtctatttgtggtcaacaccctaaacaatgtgcttattactgtgaaaataagcttcgatct

SEQ ID NO: 45 - DNA, 246 bp, ARTIFICIAL SEQUENCE
  TACI W40R, Q59R, T61P, K98T ECD
gtggcaatgcgctcatgcccagaggaacaatatcgggatccgcttcttgggacgtgtatgagctgcaagaccatctgtaatcatcaatcccgaaggccatgcgcagcattctgcaggagtctctcttgcaggaaagagcaaggcaaattttacgaccatcttttgcgagactgtataagctgtgcgtctatttgtggacaacaccctacacaatgtgcttatttctgtgaaaataagcttcgatct

SEQ ID NO: 46 - DNA, 246 bp, ARTIFICIAL SEQUENCE
  TACI L82P, I87L ECD
gtggcaatgcgctcatgcccagaggaacaatattgggatccgcttcttgggacgtgtatgagctgcaagaccatctgtaatcatcaatcccaaaggacatgcgcagctttctgcaggagtctctcttgcaggaaagagcaaggcaaattttacgaccatcctttgcgagactgtttaagctgtgcgtctatttgtggacaacaccctaaacaatgtgcttatttctgtgaaaataagcttcgatct

SEQ ID NO: 47 - DNA, 246 bp, ARTIFICIAL SEQUENCE
  TACI G76S, P97S ECD
gtggcaatgcgctcatgcccagaggaacaatattgggatccgcttcttgggacgtgtatgagctgcaagaccatctgtaatcatcaatcccaaaggacatgcgcagctttctgcaggagtctctcttgcaggaaagagcaaagcaaattttacgaccatcttttgcgagactgtataagctgtgcgtctatttgtggtcaacactctaaacaatgtgcttatttctgtgaaaataagcttcgatct

SEQ ID NO: 48 - DNA, 129 bp, ARTIFICIAL SEQUENCE
  TACI WT ECD
agtctctcttgcaggaaagagcaaggcaaattttacgaccatcttttgcgagactgtataagctgtgcgtctatttgtggacaacaccctaaacaatgtgcttatttctgtgaaaataagcttcgatct

SEQ ID NO: 49 - DNA, 129 bp, ARTIFICIAL SEQUENCE
  TACI D85V ECD
agtctctcttgcaggaaagagcaaggcaaattttacgaccatcttttgcgagtctgtataagctgtgcgtctatttgtggacaacaccctaaacaatgtgcttatttctgtgaaaataagcttcgatct

SEQ ID NO: 50 - DNA, 129 bp, ARTIFICIAL SEQUENCE
  TACI E74V ECD
agtctctcttgcaggaaagtgcaaggcaaattttacgaccatcttttgcgagactgtataagctgtgcgtctatttgtggacaacaccctaaacaatgtgcttatttctgtgaaaataagcttcgatct

SEQ ID NO: 51 - DNA, 129 bp, ARTIFICIAL SEQUENCE
  TACI R84L ECD
agtctctcttgcaggaaagagcaaggcaaattttacgaccatcttttgctagactgtataagctgtgcgtctatttgtggacaacaccctaaacaatgtgcttatttctgtgaaaataagcttcgatct

SEQ ID NO: 52 - DNA, 129 bp, ARTIFICIAL SEQUENCE
  TACI K77E, R84L, F103Y ECD
agtctctcttgcaggaaagagcaaggcgaattttacgaccatcttttgctagactgtataagctgtgcgtctatttgtggacaacaccctaaacaatgtgcttattactgtgaaaataagcttcgatct

SEQ ID NO: 53 - DNA, 129 bp, ARTIFICIAL SEQUENCE
  TACI Y79F, Q99E ECD
agtctctcttgcaggaaagagcaaggcaaatttttcgaccatcttttgcgagactgtataagctgtgcgtctatttgtggacaacaccctaaagaatgtgcttatttctgtgaaaataagcttcgatct

SEQ ID NO: 54 - DNA, 129 bp, ARTIFICIAL SEQUENCE
  TACI Y79F ECD
agtctctcttgcaggaaagagcaaggcaaatttttcgaccatcttttgcgagactgtataagctgtgcgtctatttgtggacaacaccctaaacaatgtgcttatttctgtgaaaataagcttcgatct

SEQ ID NO: 55 - DNA, 129 bp, ARTIFICIAL SEQUENCE
  TACI R84G ECD
agtctctcttgcaggaaagagcaaggcaaattttacgaccatcttttgggagactgtataagctgtgcgtctatttgtggacaacaccctaaacaatgtgcttatttctgtgaaaataagcttcgatct

SEQ ID NO: 56 - DNA, 246 bp, ARTIFICIAL SEQUENCE
  TACI L83S, F103S ECD
gtggcaatgcgctcatgcccagaggaacaatattgggatccgcttcttgggacgtgtatgagctgcaagaccatctgtaatcatcaatcccaaaggacatgcgcagctttctgcaggagtctctcttgcaggaaagagcaaggcaaattttacgaccatctttcgcgagactgtataagctgtgcgtctatttgtggacaacaccctaaacaatgtgcttattcctgtgaaaataagcttcgatct

SEQ ID NO: 57 - DNA, 246 bp, ARTIFICIAL SEQUENCE
  TACI L82H ECD
gtggcaatgcgctcatgcccagaggaacaatattgggatccgcttcttgggacgtgtatgagctgcaagaccatctgtaatcatcaatcccaaaggacatgcgcagctttctgcaggagtctctcttgcaggaaagagcaaggcaaattttacgaccatcatttgcgagactgtataagctgtgcgtctatctgtggacaacaccctaaacaatgtgcttatttctgtgaaaataagcttcgatct

SEQ ID NO: 58 - DNA, 129 bp, ARTIFICIAL SEQUENCE
  TACI A101D ECD
agtctctcttgcaggaaagagcaaggcaaattttacgaccatcttttgcgagactgtataagctgtgcgtctatttgtggacaacaccctaaacaatgtgattatttctgtgaaaataagcttcgatct

SEQ ID NO: 59 - DNA, 129 bp, ARTIFICIAL SEQUENCE
  TACI K77E, R84Q ECD
agtctctcttgcaggaaagagcaaggcgaattttacgaccatcttttgcaagactgtataagctgtgcgtctatttgtggacaacaccctaaacaatgtgcttatttctgtgaaaataagcttcgatct

SEQ ID NO: 60 - DNA, 129 bp, ARTIFICIAL SEQUENCE
  TACI K77E, A101D ECD
agtctctcttgcaggaaagagcaaggcgaattttacgaccatcttttgcgagactgtataagctgtgcgtctatttgtggacaacaccctaaacaatgtgattatttctgtgaaaataagcttcgatct

SEQ ID NO: 61 - DNA, 129 bp, ARTIFICIAL SEQUENCE
  TACI K77E, F78Y, Y102D ECD
agtctctcttgcaggaaagagcaaggcgaatattacgaccatcttttgcgagactgtataagctgtgcgtctatttgtggacaacaccctaaacaatgtgctgatttctgtgaaaataagcttcgatct

SEQ ID NO: 62 - DNA, 129 bp, ARTIFICIAL SEQUENCE
  TACI Q75E, R84Q ECD
agtctctcttgcaggaaagaggaaggcaaattttacgaccatcttttgcaagactgtataagctgtgcgtctatttgtggacaacaccctaaacaatgtgcttatttctgtgaaaataagcttcgatct

SEQ ID NO: 63 - DNA, 129 bp, ARTIFICIAL SEQUENCE
  TACI Q75R, R84G, I92V ECD
agtctctcttgcaggaaagagcgaggcaaattttacgaccatcttttgggagactgtataagctgtgcgtctgtttgtggacaacaccctaaacaatgtgcttatttctgtgaaaataagcttcgatct

SEQ ID NO: 64 - DNA, 129 bp, ARTIFICIAL SEQUENCE
  TACI K77E, A101D, Y102D ECD
agtctctcttgcaggaaagagcaaggcgaattttacgaccatcttttgcgagactgtataagctgtgcgtctatttgtggacaacaccctaaacaatgtgatgatttctgtgaaaataagcttcgatct

SEQ ID NO: 65 - DNA, 129 bp, ARTIFICIAL SEQUENCE
  TACI R84Q ECD
agtctctcttgcaggaaagagcaaggcaaattttatgaccatcttttgcaagactgtataagctgtgcgtctatttgtggacaacaccctaaacaatgtgcttatttctgtgaaaataagcttcgatct

SEQ ID NO: 66 - DNA, 129 bp, ARTIFICIAL SEQUENCE
  TACI R84Q, S88N, A101D ECD
agtctctcttgcaggaaagagcaaggcaaattttacgaccatcttttgcaagactgtataaactgtgcgtctatatgtggacaacaccctaaacaatgtgattatttctgtgaaaataagcttcgatct

SEQ ID NO: 67 - DNA, 129 bp, ARTIFICIAL SEQUENCE
  TACI K77E ECD
agtctctcttgcaggaaagagcaaggcgaattttacgaccatcttttgcgagactgtataagctgtgcgtctatttgtggacaacaccctaaacaatgtgcttatttctgtgaaaataagcttcgatct

SEQ ID NO: 68 - DNA, 129 bp, ARTIFICIAL SEQUENCE
  TACI R84Q, F103V ECD
agtctctcttgcaggaaagagcaaggcaaattttacgaccatcttttgcaagactgtataagctgtgcgtctatttgtggacaacaccctaaacaatgtgcttatgtctgtgaaaataagcttcgatct

SEQ ID NO: 69 - DNA, 129 bp, ARTIFICIAL SEQUENCE
  TACI K77E, Q95R, A101D ECD
agtctctcttgcaggaaagagcaaggcgaattttacgaccatcttttgcgagactgtataagctgtgcgtctatttgtggacgacaccctaaacaatgtgattatttctgtgaaaataagcttcgatct

SEQ ID NO: 70 - DNA, 129 bp, ARTIFICIAL SEQUENCE
  TACI I87M, A101D ECD
agtctctcttgcaggaaagagcaaggcaaattttacgaccatcttttgcgagactgtatgagctgtgcgtcaatttgtggacaacaccctaaacaatgtgattatttctgtgaaaataagcttcgatct

SEQ ID NO: 71 - protein, 232 aa, ARTIFICIAL SEQUENCE
  IgG1 Fc
EPKSCDKTHTCPPCPAPELLGGPSVFLFPPKPKDTLMISRTPEVTCVVVDVSHEDPEVKFNWYVDGVEVHNAKTKPREEQYNSTYRVVSVLTVLHQDWLNGKEYKCKVSNKALPAPIEKTISKAKGQPREPQVYTLPPSREEMTKNQVSLTCLVKGFYPSDIAVEWESNGQPENNYKTTPPVLDSDGSFFLYSKLTVDKSRWQQGNVFSCSVMHEALHNHYTQKSLSLSPGK

SEQ ID NO: 72 - protein, 8 aa, ARTIFICIAL SEQUENCE
  FLAG-tag
DYKDDDDK

SEQ ID NO: 73 - protein, 231 aa, ARTIFICIAL SEQUENCE
  Fc C220S/L234A/L235E/G237A/K447del
EPKSSDKTHTCPPCPAPEAEGAPSVFLFPPKPKDTLMISRTPEVTCVVVDVSHEDPEVKFNWYVDGVEVHNAKTKPREEQYNSTYRVVSVLTVLHQDWLNGKEYKCKVSNKALPAPIEKTISKAKGQPREPQVYTLPPSRDELTKNQVSLTCLVKGFYPSDIAVEWESNGQPENNYKTTPPVLDSDGSFFLYSKLTVDKSRWQQGNVFSCSVMHEALHNHYTQKSLSLSPG

SEQ ID NO: 74 - protein, 7 aa, ARTIFICIAL SEQUENCE
  Linker
GSGGGGS

SEQ ID NO: 75 - protein, 232 aa, ARTIFICIAL SEQUENCE
  Fc C220S/L234A/L235E/G237A/E356D/M358L
EPKSSDKTHTCPPCPAPEAEGAPSVFLFPPKPKDTLMISRTPEVTCVVVDVSHEDPEVKFNWYVDGVEVHNAKTKPREEQYNSTYRVVSVLTVLHQDWLNGKEYKCKVSNKALPAPIEKTISKAKGQPREPQVYTLPPSRDELTKNQVSLTCLVKGFYPSDIAVEWESNGQPENNYKTTPPVLDSDGSFFLYSKLTVDKSRWQQGNVFSCSVMHEALHNHYTQKSLSLSPGK

SEQ ID NO: 76 - protein, 5 aa, ARTIFICIAL SEQUENCE
  Linker
GSGGS

SEQ ID NO: 77 - protein, 5 aa, ARTIFICIAL SEQUENCE
  LINKER
GGGGS

SEQ ID NO: 78 - protein, 10 aa, ARTIFICIAL SEQUENCE
  LINKER
GGGGSGGGGS

SEQ ID NO: 79 - protein, 15 aa, ARTIFICIAL SEQUENCE
  LINKER
GGGGSGGGGSGGGGS

SEQ ID NO: 80 - protein, 7 aa, ARTIFICIAL SEQUENCE
  LINKER
GGGGSSA

SEQ ID NO: 81 - protein, 231 aa, ARTIFICIAL SEQUENCE
  Fc (E356D and M358L)
EPKSSDKTHTCPPCPAPELLGGPSVFLFPPKPKDTLMISRTPEVTCVVVDVSHEDPEVKFNWYVDGVEVHNAKTKPREEQYNSTYRVVSVLTVLHQDWLNGKEYKCKVSNKALPAPIEKTISKAKGQPREPQVYTLPPSRDELTKNQVSLTCLVKGFYPSDIAVEWESNGQPENNYKTTPPVLDSDGSFFLYSKLTVDKSRWQQGNVFSCSVMHEALHNHYTQKSLSLSPG

SEQ ID NO: 82 - protein, 232 aa, ARTIFICIAL SEQUENCE
  Fc (C5S (C220S), R77C, (R292C),  N82G (N297G), V87C (V302C))
EPKSSDKTHTCPPCPAPELLGGPSVFLFPPKPKDTLMISRTPEVTCVVVDVSHEDPEVKFNWYVDGVEVHNAKTKPCEEQYGSTYRCVSVLTVLHQDWLNGKEYKCKVSNKALPAPIEKTISKAKGQPREPQVYTLPPSREEMTKNQVSLTCLVKGFYPSDIAVEWESNGQPENNYKTTPPVLDSDGSFFLYSKLTVDKSRWQQGNVFSCSVMHEALHNHYTQKSLSLSPGK

SEQ ID NO: 83 - protein, 232 aa, ARTIFICIAL SEQUENCE
  Fc with C220S/L234A/L235E/G237A
EPKSSDKTHTCPPCPAPEAEGAPSVFLFPPKPKDTLMISRTPEVTCVVVDVSHEDPEVKFNWYVDGVEVHNAKTKPREEQYNSTYRVVSVLTVLHQDWLNGKEYKCKVSNKALPAPIEKTISKAKGQPREPQVYTLPPSREEMTKNQVSLTCLVKGFYPSDIAVEWESNGQPENNYKTTPPVLDSDGSFFLYSKLTVDKSRWQQGNVFSCSVMHEALHNHYTQKSLSLSPGK

SEQ ID NO: 84 - protein, 20 aa, ARTIFICIAL SEQUENCE
  LINKER
GGGGSGGGGSGGGGSGGGGS

SEQ ID NO: 85 - protein, 323 aa, ARTIFICIAL SEQUENCE
  Fc (G4S)2 TACI (516)
EPKSSDKTHTCPPCPAPEAEGAPSVFLFPPKPKDTLMISRTPEVTCVVVDVSHEDPEVKFNWYVDGVEVHNAKTKPREEQYNSTYRVVSVLTVLHQDWLNGKEYKCKVSNKALPAPIEKTISKAKGQPREPQVYTLPPSRDELTKNQVSLTCLVKGFYPSDIAVEWESNGQPENNYKTTPPVLDSDGSFFLYSKLTVDKSRWQQGNVFSCSVMHEALHNHYTQKSLSLSPGGGGGSGGGGSVAMRSCPEEQYWDPLLGTCMSCKTICNHQSQRTCAAFCRSLSCRKEQGKFYDHLLRDCISCASICGQHPKQCAYFCENKLRS

SEQ ID NO: 86 - protein, 294 aa, ARTIFICIAL SEQUENCE
  Fc (G4S)4 TACI (541)
EPKSSDKTHTCPPCPAPEAEGAPSVFLFPPKPKDTLMISRTPEVTCVVVDVSHEDPEVKFNWYVDGVEVHNAKTKPREEQYNSTYRVVSVLTVLHQDWLNGKEYKCKVSNKALPAPIEKTISKAKGQPREPQVYTLPPSRDELTKNQVSLTCLVKGFYPSDIAVEWESNGQPENNYKTTPPVLDSDGSFFLYSKLTVDKSRWQQGNVFSCSVMHEALHNHYTQKSLSLSPGGGGGSGGGGSGGGGSGGGGSSLSCRKEQGEYYDHLLRDCISCASICGQHPKQCADFCENKLRS

SEQ ID NO: 87 - protein, 30 aa, ARTIFICIAL SEQUENCE
  LINKER
EAAAKEAAAKEAAAKEAAAKEAAAKEAAAK

SEQ ID NO: 88 - protein, 293 aa, ARTIFICIAL SEQUENCE
  FULL LENGTH TACI
MSGLGRSRRGGRSRVDQEERFPQGLWTGVAMRSCPEEQYWDPLLGTCMSCKTICNHQSQRTCAAFCRSLSCRKEQGKFYDHLLRDCISCASICGQHPKQCAYFCENKLRSPVNLPPELRRQRSGEVENNSDNSGRYQGLEHRGSEASPALPGLKLSADQVALVYSTLGLCLCAVLCCFLVAVACFLKKRGDPCSCQPRSRPRQSPAKSSQDHAMEAGSPVSTSPEPVETCSFCFPECRAPTQESAVTPGTPDPTCAGRWGCHTRTTVLQPCPHIPDSGLGIVCVPAQEGGPGA

SEQ ID NO: 89 - protein, 230 aa, ARTIFICIAL SEQUENCE
  Fc K S139C, D141E, L143M, T151W
EPKSSDKTHTCPPCPAPEAEGAPSVFLFPPKPKDTLMISRTPEVTCVVVDVSHEDPEVKFNWYVDGVEVHNAKTKPREEQYNSTYRVVSVLTVLHQDWLNGKEYKCKVSNKALPAPIEKTISKAKGQPREPQVYTLPPCREEMTKNQVSLWCLVKGFYPSDIAVEWESNGQPENNYKTTPPVLDSDGSFFLYSKLTVDKSRWQQGNVFSCSVMHEALHNHYTQKSLSLSP

SEQ ID NO: 90 - protein, 230 aa, ARTIFICIAL SEQUENCE
  Fc H Y134C, D141E, L143M, T151S, L153A
EPKSSDKTHTCPPCPAPEAEGAPSVFLFPPKPKDTLMISRTPEVTCVVVDVSHEDPEVKFNWYVDGVEVHNAKTKPREEQYNSTYRVVSVLTVLHQDWLNGKEYKCKVSNKALPAPIEKTISKAKGQPREPQVCTLPPSREEMTKNQVSLSCAVKGFYPSDIAVEWESNGQPENNYKTTPPVLDSDGSFFLVSKLTVDKSRWQQGNVFSCSVMHEALHNHYTQKSLSLSP

SEQ ID NO: 91 - protein, 25 aa, ARTIFICIAL SEQUENCE
  LINKER
GGGGSGGGGSGGGGSGGGGSGGGGS

SEQ ID NO: 92 - protein, 43 aa, ARTIFICIAL SEQUENCE
  TACI L82P ECD
SLSCRKEQGKFYDHPLRDCISCASICGQHPKQCAYFCENKLRS

SEQ ID NO: 93 - protein, 43 aa, ARTIFICIAL SEQUENCE
  TACI D85E, K98T ECD
SLSCRKEQGKFYDHLLRECISCASICGQHPTQCAYFCENKLRS

SEQ ID NO: 94 - protein, 43 aa, ARTIFICIAL SEQUENCE
  TACI I87L, K98T ECD
SLSCRKEQGKFYDHLLRDCLSCASICGQHPTQCAYFCENKLRS

SEQ ID NO: 95 - protein, 43 aa, ARTIFICIAL SEQUENCE; identical to SEQ ID NO: 23
  TACI A101D ECD

SEQ ID NO: 96 - protein, 43 aa, ARTIFICIAL SEQUENCE
  TACI C86Y ECD
SLSCRKEQGKFYDHLLRDYISCASICGQHPKQCAYFCENKLRS

SEQ ID NO: 97 - protein, 43 aa, ARTIFICIAL SEQUENCE
  TACI L82P, I87L ECD
SLSCRKEQGKFYDHPLRDCLSCASICGQHPKQCAYFCENKLRS

SEQ ID NO: 98 - protein, 43 aa, ARTIFICIAL SEQUENCE
  TACI G76S, P97S ECD
SLSCRKEQSKFYDHLLRDCISCASICGQHSKQCAYFCENKLRS

SEQ ID NO: 99 - protein, 43 aa, ARTIFICIAL SEQUENCE
  TACI L83S, F103S ECD
SLSCRKEQGKFYDHLSRDCISCASICGQHPKQCAYSCENKLRS

SEQ ID NO: 100 - protein, 43 aa, ARTIFICIAL SEQUENCE
  TACI L82H ECD
SLSCRKEQGKFYDHHLRDCISCASICGQHPKQCAYFCENKLRS

SEQ ID NO: 101 - protein, 82 aa, ARTIFICIAL SEQUENCE
  TACI D85V ECD
VAMRSCPEEQYWDPLLGTCMSCKTICNHQSQRTCAAFCRSLSCRKEQGKFYDHLLRVCISCASICGQHPKQCAYFCENKLRS

SEQ ID NO: 102 - protein, 82 aa, ARTIFICIAL SEQUENCE
  TACI E74V ECD
VAMRSCPEEQYWDPLLGTCMSCKTICNHQSQRTCAAFCRSLSCRKVQGKFYDHLLRDCISCASICGQHPKQCAYFCENKLRS

SEQ ID NO: 103 - protein, 82 aa, ARTIFICIAL SEQUENCE
  TACI R84L ECD
VAMRSCPEEQYWDPLLGTCMSCKTICNHQSQRTCAAFCRSLSCRKEQGKFYDHLLLDCISCASICGQHPKQCAYFCENKLRS

SEQ ID NO: 104 - protein, 82 aa, ARTIFICIAL SEQUENCE
  TACI K77E, R84L, F103Y ECD
VAMRSCPEEQYWDPLLGTCMSCKTICNHQSQRTCAAFCRSLSCRKEQGEFYDHLLLDCISCASICGQHPKQCAYYCENKLRS

SEQ ID NO: 105 - protein, 82 aa, ARTIFICIAL SEQUENCE
  TACI Y79F, Q99E ECD
VAMRSCPEEQYWDPLLGTCMSCKTICNHQSQRTCAAFCRSLSCRKEQGKFFDHLLRDCISCASICGQHPKECAYFCENKLRS

SEQ ID NO: 106 - protein, 82 aa, ARTIFICIAL SEQUENCE
  TACI Y79F ECD
VAMRSCPEEQYWDPLLGTCMSCKTICNHQSQRTCAAFCRSLSCRKEQGKFFDHLLRDCISCASICGQHPKQCAYFCENKLRS

SEQ ID NO: 107 - protein, 82 aa, ARTIFICIAL SEQUENCE
  TACI R84G ECD
VAMRSCPEEQYWDPLLGTCMSCKTICNHQSQRTCAAFCRSLSCRKEQGKFYDHLLGDCISCASICGQHPKQCAYFCENKLRS

SEQ ID NO: 108 - protein, 82 aa, ARTIFICIAL SEQUENCE; identical to SEQ ID NO: 7
  TACI A101D ECD

SEQ ID NO: 109 - protein, 82 aa, ARTIFICIAL SEQUENCE
  TACI K77E, R84Q ECD
VAMRSCPEEQYWDPLLGTCMSCKTICNHQSQRTCAAFCRSLSCRKEQGEFYDHLLQDCISCASICGQHPKQCAYFCENKLRS

SEQ ID NO: 110 - protein, 82 aa, ARTIFICIAL SEQUENCE
  TACI K77E, A101D ECD
VAMRSCPEEQYWDPLLGTCMSCKTICNHQSQRTCAAFCRSLSCRKEQGEFYDHLLRDCISCASICGQHPKQCDYFCENKLRS

SEQ ID NO: 111 - protein, 82 aa, ARTIFICIAL SEQUENCE
  TACI K77E, F78Y, Y102D ECD
VAMRSCPEEQYWDPLLGTCMSCKTICNHQSQRTCAAFCRSLSCRKEQGEYYDHLLRDCISCASICGQHPKQCADFCENKLRS

SEQ ID NO: 112 - protein, 82 aa, ARTIFICIAL SEQUENCE
  TACI Q75E, R84Q ECD
VAMRSCPEEQYWDPLLGTCMSCKTICNHQSQRTCAAFCRSLSCRKEEGKFYDHLLQDCISCASICGQHPKQCAYFCENKLRS

SEQ ID NO: 113 - protein, 82 aa, ARTIFICIAL SEQUENCE
  TACI Q75R, R84G, I92V ECD
VAMRSCPEEQYWDPLLGTCMSCKTICNHQSQRTCAAFCRSLSCRKERGKFYDHLLGDCISCASVCGQHPKQCAYFCENKLRS

SEQ ID NO: 114 - protein, 82 aa, ARTIFICIAL SEQUENCE
  TACI K77E, A101D, Y102D ECD
VAMRSCPEEQYWDPLLGTCMSCKTICNHQSQRTCAAFCRSLSCRKEQGEFYDHLLRDCISCASICGQHPKQCDDFCENKLRS

SEQ ID NO: 115 - protein, 82 aa, ARTIFICIAL SEQUENCE
  TACI R84Q ECD
VAMRSCPEEQYWDPLLGTCMSCKTICNHQSQRTCAAFCRSLSCRKEQGKFYDHLLQDCISCASICGQHPKQCAYFCENKLRS

SEQ ID NO: 116 - protein, 82 aa, ARTIFICIAL SEQUENCE
  TACI R84Q, S88N, A101D ECD
VAMRSCPEEQYWDPLLGTCMSCKTICNHQSQRTCAAFCRSLSCRKEQGKFYDHLLQDCINCASICGQHPKQCDYFCENKLRS

SEQ ID NO: 117 - protein, 82 aa, ARTIFICIAL SEQUENCE
  TACI K77E ECD
VAMRSCPEEQYWDPLLGTCMSCKTICNHQSQRTCAAFCRSLSCRKEQGEFYDHLLRDCISCASICGQHPKQCAYFCENKLRS

SEQ ID NO: 118 - protein, 82 aa, ARTIFICIAL SEQUENCE
  TACI R84Q, F103V ECD
VAMRSCPEEQYWDPLLGTCMSCKTICNHQSQRTCAAFCRSLSCRKEQGKFYDHLLQDCISCASICGQHPKQCAYVCENKLRS

SEQ ID NO: 119 - protein, 82 aa, ARTIFICIAL SEQUENCE
  TACI K77E, Q95R, A101D ECD
VAMRSCPEEQYWDPLLGTCMSCKTICNHQSQRTCAAFCRSLSCRKEQGEFYDHLLRDCISCASICGRHPKQCDYFCENKLRS

SEQ ID NO: 120 - protein, 82 aa, ARTIFICIAL SEQUENCE
  TACI I87M, A101D ECD
VAMRSCPEEQYWDPLLGTCMSCKTICNHQSQRTCAAFCRSLSCRKEQGKFYDHLLRDCMSCASICGQHPKQCDYFCENKLRS

SEQ ID NO: 121 - protein, 660 aa, ARTIFICIAL SEQUENCE
  CTLA4 113 GSG4S Fc K/ BCMA 357 GSG4S Fc H
KAMHVAQPAVVFASSHGIASFVCEYASPWKATEVRVTVLRQADSQVTEVCAATYMTGNELTFLDDSICTGTSSGNQVNLTIQGLRAMDTGLYICKVEQMYPPPYLLGIGNGTQIYVIDPEPCPDSDGSGGGGSEPKSSDKTHTCPPCPAPEAEGAPSVFLFPPKPKDTLMISRTPEVTCVVVDVSHEDPEVKFNWYVDGVEVHNAKTKPREEQYNSTYRVVSVLTVLHQDWLNGKEYKCKVSNKALPAPIEKTISKAKGQPREPQVYTLPPCREEMTKNQVSLWCLVKGFYPSDIAVEWESNGQPENNYKTTPPVLDSDGSFFLYSKLTVDKSRWQQGNVFSCSVMHEALHNHYTQKSLSLSPGLQMAGQCSQNEYFDSLLYACIPCQLRCSSNTPPLTCQRYCNASVTNSVKGTNAGSGGSGGSGGSGSEPKSSDKTHTCPPCPAPEAEGAPSVFLFPPKPKDTLMISRTPEVTCVVVDVSHEDPEVKFNWYVDGVEVHNAKTKPREEQYNSTYRVVSVLTVLHQDWLNGKEYKCKVSNKALPAPIEKTISKAKGQPREPQVCTLPPSREEMTKNQVSLSCAVKGFYPSDIAVEWESNGQPENNYKTTPPVLDSDGSFFLVSKLTVDKSRWQQGNVFSCSVMHEALHNHYTQKSLSLSP

SEQ ID NO: 122 - protein, 166 aa, artificial sequence
  TACI ECD (1-166)
MSGLGRSRRGGRSRVDQEERFPQGLWTGVAMRSCPEEQYWDPLLGTCMSCKTICNHQSQRTCAAFCRSLSCRKEQGKFYDHLLRDCISCASICGQHPKQCAYFCENKLRSPVNLPPELRRQRSGEVENNSDNSGRYQGLEHRGSEASPALPGLKLSADQVALVYST

SEQ ID NO: 123 - protein, 5 aa, artificial sequence
  1xEAAAK
EAAAK

SEQ ID NO: 124 - protein, 10 aa, artificial sequence
  2xEAAAK
EAAAKEAAAK

SEQ ID NO: 125 - protein, 15 aa, artificial sequence
  3xEAAAK
EAAAKEAAAKEAAAK

SEQ ID NO: 126 - protein, 20 aa, artificial sequence
  4xEAAAK
EAAAKEAAAKEAAAKEAAAK

SEQ ID NO: 127 - protein, 25 aa, artificial sequence
  5xEAAAK
EAAAKEAAAKEAAAKEAAAKEAAAK

SEQ ID NO: 128 - protein, 232 aa, artificial sequence
  knob Fc
EPKSSDKTHTCPPCPAPEAEGAPSVFLFPPKPKDTLMISRTPEVTCVVVDVSHEDPEVKFNWYVDGVEVHNAKTKPREEQYNSTYRVVSVLTVLHQDWLNGKEYKCKVSNKALPAPIEKTISKAKGQPREPQVYTLPPCREEMTKNQVSLWCLVKGFYPSDIAVEWESNGQPENNYKTTPPVLDSDGSFFLYSKLTVDKSRWQQGNVFSCSVMHEALHNHYTQKSLSLSPGK

SEQ ID NO: 129 - protein, 232 aa, artificial sequence
  hole Fc
EPKSSDKTHTCPPCPAPEAEGAPSVFLFPPKPKDTLMISRTPEVTCVVVDVSHEDPEVKFNWYVDGVEVHNAKTKPREEQYNSTYRVVSVLTVLHQDWLNGKEYKCKVSNKALPAPIEKTISKAKGQPREPQVCTLPPSREEMTKNQVSLSCAVKGFYPSDIAVEWESNGQPENNYKTTPPVLDSDGSFFLVSKLTVDKSRWQQGNVFSCSVMHEALHNHYTQKSLSLSPGK

SEQ ID NO: 130 - protein, 81 aa, artificial sequence
  atacicept (TACI portion, 30-110)
AMRSCPEEQYWDPLLGTCMSCKTICNHQSQRTCAAFCRSLSCRKEQGKFYDHLLRDCISCASICGQHPKQCAYFCENKLRS

SEQ ID NO: 131 - protein, 106 aa, artificial sequence
  telitacicept (TACI portion, 13-118)
SRVDQEERFPQGLWTGVAMRSCPEEQYWDPLLGTCMSCKTICNHQSQRTCAAFCRSLSCRKEQGKFYDHLLRDCISCASICGQHPKQCAYFCENKLRSPVNLPPEL

SEQ ID NO: 132 - protein, 313 aa, artificial sequence
  atacicept
AMRSCPEEQYWDPLLGTCMSCKTICNHQSQRTCAAFCRSLSCRKEQGKFYDHLLRDCISCASICGQHPKQCAYFCENKLRSEPKSSDKTHTCPPCPAPEAEGAPSVFLFPPKPKDTLMISRTPEVTCVVVDVSHEDPEVKFNWYVDGVEVHNAKTKPREEQYNSTYRVVSVLTVLHQDWLNGKEYKCKVSNKALPSSIEKTISKAKGQPREPQVYTLPPSRDELTKNQVSLTCLVKGFYPSDIAVEWESNGQPENNYKTTPPVLDSDGSFFLYSKLTVDKSRWQQGNVFSCSVMHEALHNHYTQKSLSLSPGK

SEQ ID NO: 133 - protein, 13 aa, artificial sequence
  linker
GGGGSGGGGSAAA

SEQ ID NO: 134 - protein, 231 aa, artificial sequence
  Fc with C220S/E233P/L234V/L235A/G236del/S267K
EPKSSDKTHTCPPCPAPPVAGPSVFLFPPKPKDTLMISRTPEVTCVVVDVKHEDPEVKFNWYVDGVEVHNAKTKPREEQYNSTYRVVSVLTVLHQDWLNGKEYKCKVSNKALPAPIEKTISKAKGQPREPQVYTLPPSREEMTKNQVSLTCLVKGFYPSDIAVEWESNGQPENNYKTTPPVLDSDGSFFLYSKLTVDKSRWQQGNVFSCSVMHEALHNHYTQKSLSLSPGK

SEQ ID NO: 135 - protein, 231 aa, artificial sequence
  Fc (C5S (C220S), R77C, (R292C),  N82G (N297G), V87C (V302C), L232del (K447del))
EPKSSDKTHTCPPCPAPELLGGPSVFLFPPKPKDTLMISRTPEVTCVVVDVSHEDPEVKFNWYVDGVEVHNAKTKPCEEQYGSTYRCVSVLTVLHQDWLNGKEYKCKVSNKALPAPIEKTISKAKGQPREPQVYTLPPSREEMTKNQVSLTCLVKGFYPSDIAVEWESNGQPENNYKTTPPVLDSDGSFFLYSKLTVDKSRWQQGNVFSCSVMHEALHNHYTQKSLSLSPG

SEQ ID NO: 136 - protein, 231 aa, artificial sequence
  Fc with C220S/L234A/L235E/G237A/K447del
EPKSSDKTHTCPPCPAPEAEGAPSVFLFPPKPKDTLMISRTPEVTCVVVDVSHEDPEVKFNWYVDGVEVHNAKTKPREEQYNSTYRVVSVLTVLHQDWLNGKEYKCKVSNKALPAPIEKTISKAKGQPREPQVYTLPPSREEMTKNQVSLTCLVKGFYPSDIAVEWESNGQPENNYKTTPPVLDSDGSFFLYSKLTVDKSRWQQGNVFSCSVMHEALHNHYTQKSLSLSPG

SEQ ID NO: 137 - protein, 230 aa, artificial sequence
  Fc with C220S/E233P/L234V/L235A/G236del/S267K/K447del
EPKSSDKTHTCPPCPAPPVAGPSVFLFPPKPKDTLMISRTPEVTCVVVDVKHEDPEVKFNWYVDGVEVHNAKTKPREEQYNSTYRVVSVLTVLHQDWLNGKEYKCKVSNKALPAPIEKTISKAKGQPREPQVYTLPPSREEMTKNQVSLTCLVKGFYPSDIAVEWESNGQPENNYKTTPPVLDSDGSFFLYSKLTVDKSRWQQGNVFSCSVMHEALHNHYTQKSLSLSPG

SEQ ID NO: 138 - protein, 235 aa, artificial sequence
  IgG2 Fc
TKVDKTVERKCCVECPPCPAPPVAGPSVFLFPPKPKDTLMISRTPEVTCVVVDVSHEDPEVQFNWYVDGVEVHNAKTKPREEQFNSTFRVVSVLTVVHQDWLNGKEYKCKVSNKGLPAPIEKTISKTKGQPREPQVYTLPPSREEMTKNQVSLTCLVKGFYPSDIAVEWESNGQPENNYKTTPPMLDSDGSFFLYSKLTVDKSRWQQGNVFSCSVMHEALHNHYTQKSLSLSPGK

SEQ ID NO: 139 - protein, 229 aa, artificial sequence
  IgG4 Fc
ESKYGPPCPSCPAPEFLGGPSVFLFPPKPKDTLMISRTPEVTCVVVDVSQEDPEVQFNWYVDGVEVHNAKTKPREEQFNSTYRVVSVLTVLHQDWLNGKEYKCKVSNKGLPSSIEKTISKAKGQPREPQVYTLPPSQEEMTKNQVSLTCLVKGFYPSDIAVEWESNGQPENNYKTTPPVLDSDGSFFLYSRLTVDKSRWQEGNVFSCSVMHEALHNHYTQKSLSLSLGK

SEQ ID NO: 140 - protein, 229 aa, artificial sequence
  IgG4 Fc S228P
ESKYGPPCPPCPAPEFLGGPSVFLFPPKPKDTLMISRTPEVTCVVVDVSQEDPEVQFNWYVDGVEVHNAKTKPREEQFNSTYRVVSVLTVLHQDWLNGKEYKCKVSNKGLPSSIEKTISKAKGQPREPQVYTLPPSQEEMTKNQVSLTCLVKGFYPSDIAVEWESNGQPENNYKTTPPVLDSDGSFFLYSRLTVDKSRWQEGNVFSCSVMHEALHNHYTQKSLSLSLGK

SEQ ID NO: 141 - protein, 231 aa, artificial sequence
  Fc K chain
EPKSSDKTHTCPPCPAPEAEGAPSVFLFPPKPKDTLMISRTPEVTCVVVDVSHEDPEVKFNWYVDGVEVHNAKTKPREEQYNSTYRVVSVLTVLHQDWLNGKEYKCKVSNKALPAPIEKTISKAKGQPREPQVYTLPPSRKKMTKNQVSLTCLVKGFYPSDIAVEWESNGQPENNYKTTPPVLKSDGSFFLYSKLTVDKSRWQQGNVFSCSVMHEALHNHYTQKSLSLSPG

SEQ ID NO: 142 - protein, 231 aa, artificial sequence
  Fc D chain
EPKSSDKTHTCPPCPAPEAEGAPSVFLFPPKPKDTLMISRTPEVTCVVVDVSHEDPEVKFNWYVDGVEVHNAKTKPREEQYNSTYRVVSVLTVLHQDWLNGKEYKCKVSNKALPAPIEKTISKAKGQPREPQVYTLPPSREEMTKNQVSLTCLVDGFYPSDIAVEWESNGQPENNYDTTPPVLDSDGSFFLYSDLTVDKSRWQQGNVFSCSVMHEALHNHYTQKSLSLSPG

SEQ ID NO: 143 - protein, 237 aa, artificial sequence
  Green Fluorescent protein
SKGEELFTGVVPILVELDGDVNGHKFSVSGEGEGDATYGKLTLKFICTTGKLPVPWPTLVTTFSYGVQCFSRYPDHMKQHDFFKSAMPEGYVQERTIFFKDDGNYKTRAEVKFEGDTLVNRIELKGIDFKEDGNILGHKLEYNYNSHNVYIMADKQKNGIKVNFKIRHNIEDGSVQLADHYQQNTPIGDGPVLLPDNHYLSTQSALSKDPNEKRDHMVLLEFVTAAGITHGMDELYK

SEQ ID NO: 144 - protein, 237 aa, artificial sequence
  eGFP
SKGEELFTGVVPILVELDGDVNGHKFSVSGEGEGDATYGKLTLKFICTTGKLPVPWPTLVTTLTYGVQCFSRYPDHMKQHDFFKSAMPEGYVQERTIFFKDDGNYKTRAEVKFEGDTLVNRIELKGIDFKEDGNILGHKLEYNYNSHNVYIMADKQKNGIKVNFKIRHNIEDGSVQLADHYQQNTPIGDGPVLLPDNHYLSTQSALSKDPNEKRDHMVLLEFVTAAGITHGMDELYK

SEQ ID NO: 145 - protein, 239 aa, artificial sequence
  eGFP
MVSKGEELFTGVVPILVELDGDVNGHKFSVSGEGEGDATYGKLTLKFICTTGKLPVPWPTLVTTLTYGVQCFSRYPDHMKQHDFFKSAMPEGYVQERTIFFKDDGNYKTRAEVKFEGDTLVNRIELKGIDFKEDGNILGHKLEYNYNSHNVYIMADKQKNGIKVNFKIRHNIEDGSVQLADHYQQNTPIGDGPVLLPDNHYLSTQSALSKDPNEKRDHMVLLEFVTAAGITLGMDELYK

SEQ ID NO: 146 - protein, 45 aa, artificial sequence
  Moiety: COMP
DLGPQMLRELQETNAALQDVRELLRQQVREITFLKNTVMECDACG

SEQ ID NO: 147 - protein, 33 aa, artificial sequence
  Moiety: VASP
DLQRVKQELLEEVKKELQKVKEEIIEAFVQELR

SEQ ID NO: 148 - protein, 40 aa, artificial sequence
  Moiety: ZZ12.6
DVQAISSTIQDLQDQVDSLAEVVLQNRRGLDLLTRSGGGS

SEQ ID NO: 149 - protein, 18 aa, artificial sequence
  HSA signal peptide
MKWVTFISLLFLFSSAYS

SEQ ID NO: 150 - protein, 22 aa, artificial sequence
  Ig kappa light chain
MDMRAPAGIFGFLLVLFPGYRS

SEQ ID NO: 151 - protein, 19 aa, artificial sequence
  human azurocidin preprotein signal sequence
MTRLTVLALLAGLLASSRA

SEQ ID NO: 152 - protein, 19 aa, artificial sequence
  IgG heavy chain signal peptide
MELGLSWIFLLAILKGVQC

SEQ ID NO: 153 - protein, 19 aa, artificial sequence
  IgG heavy chain signal peptide
MELGLRWVFLVAILEGVQC

SEQ ID NO: 154 - protein, 19 aa, artificial sequence
  IgG heavy chain signal peptide
MKHLWFFLLLVAAPRWVLS

SEQ ID NO: 155 - protein, 19 aa, artificial sequence
  IgG heavy chain signal peptide
MDWTWRILFLVAAATGAHS

SEQ ID NO: 156 - protein, 19 aa, artificial sequence
  IgG heavy chain signal peptide
MDWTWRFLFVVAAATGVQS

SEQ ID NO: 157 - protein, 19 aa, artificial sequence
  IgG heavy chain signal peptide
MEFGLSWLFLVAILKGVQC

SEQ ID NO: 158 - protein, 19 aa, artificial sequence
  IgG heavy chain signal peptide
MEFGLSWVFLVALFRGVQC

SEQ ID NO: 159 - protein, 26 aa, artificial sequence
  IgG heavy chain signal peptide
MDLLHKNMKHLWFFLLLVAAPRWVLS

SEQ ID NO: 160 - protein, 22 aa, artificial sequence
  IgG Kappa light chain signal sequence
MDMRVPAQLLGLLLLWLSGARC

SEQ ID NO: 161 - protein, 22 aa, artificial sequence
  IgG Kappa light chain signal sequence
MKYLLPTAAAGLLLLAAQPAMA

SEQ ID NO: 162 - protein, 17 aa, artificial sequence
  Gaussia luciferase
MGVKVLFALICIAVAEA

SEQ ID NO: 163 - protein, 18 aa, homo sapiens
  MISC_FEATURE: Human albumin
MKWVTFISLLFLFSSAYS

SEQ ID NO: 164 - protein, 18 aa, homo sapiens
  MISC_FEATURE: Human chymotrypsinogen
MAFLWLLSCWALLGTTFG

SEQ ID NO: 165 - protein, 14 aa, homo sapiens
  MISC_FEATURE: Human interleukin-2
MQLLSCIALILALV

SEQ ID NO: 166 - protein, 15 aa, homo sapiens
  MISC_FEATURE: Human trypsinogen-2
MNLLLILTFVAAAVA

SEQ ID NO: 167 - protein, 281 aa, artificial sequence
  TACI Fc
SLSCRKEQGEYYDHLLRDCISCASICGQHPKQCADFCENKLRSGSGGGGSEPKSSDKTHTCPPCPAPEAEGAPSVFLFPPKPKDTLMISRTPEVTCVVVDVSHEDPEVKFNWYVDGVEVHNAKTKPREEQYNSTYRVVSVLTVLHQDWLNGKEYKCKVSNKALPAPIEKTISKAKGQPREPQVYTLPPSRDELTKNQVSLTCLVKGFYPSDIAVEWESNGQPENNYKTTPPVLDSDGSFFLYSKLTVDKSRWQQGNVFSCSVMHEALHNHYTQKSLSLSPG

SEQ ID NO: 168 - protein, 281 aa, artificial sequence
  TACI Fc
SLSCRKEQGEYYDHLLRDCISCASICGQHPKQCADFCENKLRSGSGGGGSEPKSSDKTHTCPPCPAPELLGGPSVFLFPPKPKDTLMISRTPEVTCVVVDVSHEDPEVKFNWYVDGVEVHNAKTKPREEQYNSTYRVVSVLTVLHQDWLNGKEYKCKVSNKALPAPIEKTISKAKGQPREPQVYTLPPSRDELTKNQVSLTCLVKGFYPSDIAVEWESNGQPENNYKTTPPVLDSDGSFFLYSKLTVDKSRWQQGNVFSCSVMHEALHNHYTQKSLSLSPG

SEQ ID NO: 169 - protein, 281 aa, artificial sequence
  TACI Fc
SLSCRKEEGKFYDHLLQDCISCASICGQHPKQCAYFCENKLRSGSGGGGSEPKSSDKTHTCPPCPAPEAEGAPSVFLFPPKPKDTLMISRTPEVTCVVVDVSHEDPEVKFNWYVDGVEVHNAKTKPREEQYNSTYRVVSVLTVLHQDWLNGKEYKCKVSNKALPAPIEKTISKAKGQPREPQVYTLPPSRDELTKNQVSLTCLVKGFYPSDIAVEWESNGQPENNYKTTPPVLDSDGSFFLYSKLTVDKSRWQQGNVFSCSVMHEALHNHYTQKSLSLSPG

SEQ ID NO: 170 - protein, 281 aa, artificial sequence
  TACI Fc
SLSCRKEEGKFYDHLLQDCISCASICGQHPKQCAYFCENKLRSGSGGGGSEPKSSDKTHTCPPCPAPELLGGPSVFLFPPKPKDTLMISRTPEVTCVVVDVSHEDPEVKFNWYVDGVEVHNAKTKPREEQYNSTYRVVSVLTVLHQDWLNGKEYKCKVSNKALPAPIEKTISKAKGQPREPQVYTLPPSRDELTKNQVSLTCLVKGFYPSDIAVEWESNGQPENNYKTTPPVLDSDGSFFLYSKLTVDKSRWQQGNVFSCSVMHEALHNHYTQKSLSLSPG

SEQ ID NO: 171 - protein, 281 aa, artificial sequence
  TACI Fc
SLSCRKEQGKFYDHLLRDCISCASICGQHPKQCAYFCENKLRSGSGGGGSEPKSSDKTHTCPPCPAPEAEGAPSVFLFPPKPKDTLMISRTPEVTCVVVDVSHEDPEVKFNWYVDGVEVHNAKTKPREEQYNSTYRVVSVLTVLHQDWLNGKEYKCKVSNKALPAPIEKTISKAKGQPREPQVYTLPPSRDELTKNQVSLTCLVKGFYPSDIAVEWESNGQPENNYKTTPPVLDSDGSFFLYSKLTVDKSRWQQGNVFSCSVMHEALHNHYTQKSLSLSPG

SEQ ID NO: 172 - protein, 281 aa, artificial sequence
  TACI Fc
SLSCRKEQGKFYDHLLRDCISCASICGQHPKQCAYFCENKLRSGSGGGGSEPKSSDKTHTCPPCPAPELLGGPSVFLFPPKPKDTLMISRTPEVTCVVVDVSHEDPEVKFNWYVDGVEVHNAKTKPREEQYNSTYRVVSVLTVLHQDWLNGKEYKCKVSNKALPAPIEKTISKAKGQPREPQVYTLPPSRDELTKNQVSLTCLVKGFYPSDIAVEWESNGQPENNYKTTPPVLDSDGSFFLYSKLTVDKSRWQQGNVFSCSVMHEALHNHYTQKSLSLSPG

SEQ ID NO: 173 - protein, 227 aa, artificial sequence
  Fc
DKPHTCPLCPAPELLGGPSVFLFPPKPKDTLMISRTPEVTCVVVDVSHEDPEVKFNWYVDGVEVHNAKTKPREEQYNSTYRVVSVLTVLHQDWLNGKEYKCKVSNKALPAPIEKTISKAKGQPREPQVYTLPPSRDELTKNQVSLTCLVKGFYPSDIAVEWESNGQPENNYKATPPVLDSDGSFFLYSKLTVDKSRWQQGNVFSCSVMHEALHNHYTQKSLSLSPGK

SEQ ID NO: 174 - protein, 232 aa, artificial sequence
  Fc
DPKSCDKPHTCPLCPAPELLGGPSVFLFPPKPKDTLMISRTPEVTCVVVDVSHEDPEVKFNWYVDGVEVHNAKTKPREEQYNSTYRVVSVLTVLHQDWLNGKEYKCKVSNKALPAPIEKTISKAKGQPREPQVYTLPPSRDELTKNQVSLTCLVKGFYPSDIAVEWESNGQPENNYKATPPVLDSDGSFFLYSKLTVDKSRWQQGNVFSCSVMHEALHNHYTQKSLSLSPGK

SEQ ID NO: 175 - protein, 227 aa, artificial sequence
  Fc variant
DKTHTCPPCPAPEAEGAPSVFLFPPKPKDTLMISRTPEVTCVVVDVSHEDPEVKFNWYVDGVEVHNAKTKPREEQYNSTYRVVSVLTVLHQDWLNGKEYKCKVSNKALPSSIEKTISKAKGQPREPQVYTLPPSRDELTKNQVSLTCLVKGFYPSDIAVEWESNGQPENNYKTTPPVLDSDGSFFLYSKLTVDKSRWQQGNVFSCSVMHEALHNHYTQKSLSLSPGK

SEQ ID NO: 176 - protein, 232 aa, artificial sequence
  Fc variant
EPKSSDKTHTCPPCPAPEAEGAPSVFLFPPKPKDTLMISRTPEVTCVVVDVSHEDPEVKFNWYVDGVEVHNAKTKPREEQYNSTYRVVSVLTVLHQDWLNGKEYKCKVSNKALPSSIEKTISKAKGQPREPQVYTLPPSRDELTKNQVSLTCLVKGFYPSDIAVEWESNGQPENNYKTTPPVLDSDGSFFLYSKLTVDKSRWQQGNVFSCSVMHEALHNHYTQKSLSLSPGK

SEQ ID NO: 177 - protein, 43 aa, artificial sequence
  TACI variant
SLSCRKEEGKFYDHLLRDCISCASICGQHPKQCAYFCENKLRS

SEQ ID NO: 178 - protein, 43 aa, artificial sequence
  TACI variant
SLSCRKEEGEFYDHLLRDCISCASICGQHPKQCAYFCENKLRS

SEQ ID NO: 179 - protein, 43 aa, artificial sequence
  TACI variant
SLSCRKEEGKYYDHLLRDCISCASICGQHPKQCAYFCENKLRS

SEQ ID NO: 180 - protein, 43 aa, artificial sequence
  TACI variant
SLSCRKEEGKFYDHLLRDCISCASICGQHPKQCDYFCENKLRS

SEQ ID NO: 181 - protein, 43 aa, artificial sequence
  TACI variant
SLSCRKEEGKFYDHLLRDCISCASICGQHPKQCADFCENKLRS

SEQ ID NO: 182 - protein, 43 aa, artificial sequence
  TACI variant
SLSCRKEQGEYYDHLLQDCISCASICGQHPKQCAYFCENKLRS

SEQ ID NO: 183 - protein, 43 aa, artificial sequence
  TACI variant
SLSCRKEQGKYYDHLLRDCISCASICGQHPKQCAYFCENKLRS

SEQ ID NO: 184 - protein, 43 aa, artificial sequence
  TACI variant
SLSCRKEQGKYYDHLLQDCISCASICGQHPKQCAYFCENKLRS

SEQ ID NO: 185 - protein, 43 aa, artificial sequence
  TACI variant
SLSCRKEQGKYYDHLLRDCISCASICGQHPKQCDYFCENKLRS

SEQ ID NO: 186 - protein, 43 aa, artificial sequence
  TACI variant
SLSCRKEQGKYYDHLLRDCISCASICGQHPKQCADFCENKLRS

SEQ ID NO: 187 - protein, 43 aa, artificial sequence
  TACI variant
SLSCRKEQGKFYDHLLQDCISCASICGQHPKQCDYFCENKLRS

SEQ ID NO: 188 - protein, 43 aa, artificial sequence
  TACI variant
SLSCRKEQGKFYDHLLQDCISCASICGQHPKQCADFCENKLRS

SEQ ID NO: 189 - protein, 43 aa, artificial sequence
  TACI variant
SLSCRKEQGKFYDHLLRDCISCASICGQHPKQCDDFCENKLRS

SEQ ID NO: 190 - protein, 43 aa, artificial sequence
  TACI variant
SLSCRKEQGKFYDHLLRDCISCASICGQHPKQCADFCENKLRS

SEQ ID NO: 191 - protein, 43 aa, artificial sequence
  TACI variant
SLSCRKEQGEYYDHLLRDCISCASICGQHPKQCAYFCENKLRS

SEQ ID NO: 192 - protein, 43 aa, artificial sequence
  TACI variant
SLSCRKEQGEFYDHLLRDCISCASICGQHPKQCADFCENKLRS

SEQ ID NO: 193 - protein, 227 aa, artificial sequence; identical to SEQ ID NO: 173
  Fc variant

SEQ ID NO: 194 - protein, 12 aa, artificial sequence
  linker
GSGGGGSGGGGS

SEQ ID NO: 195 - protein, 65 aa, artificial sequence
  linker
GGGGSGGGGSGGGGSGGGGSGGGGSGGGGSGGGGSGGGGSGGGGSGGGGSGGGGSGGGGSGGGGS

SEQ ID NO: 196 - protein, 577 aa, artificial sequence
  TACI FC
SLSCRKEQGKFYDHLLRDCISCASICGQHPKQCAYFCENKLRSGSGGGGSGGGGSEPKSSDKTHTCPPCPAPEAEGAPSVFLFPPKPKDTLMISRTPEVTCVVVDVSHEDPEVKFNWYVDGVEVHNAKTKPREEQYNSTYRVVSVLTVLHQDWLNGKEYKCKVSNKALPAPIEKTISKAKGQPREPQVYTLPPSRDELTKNQVSLTCLVKGFYPSDIAVEWESNGQPENNYKTTPPVLDSDGSFFLYSKLTVDKSRWQQGNVFSCSVMHEALHNHYTQKSLSLSPGGGGGSGGGGSGGGGSGGGGSGGGGSGGGGSGGGGSGGGGSGGGGSGGGGSGGGGSGGGGSEPKSSDKTHTCPPCPAPEAEGAPSVFLFPPKPKDTLMISRTPEVTCVVVDVSHEDPEVKFNWYVDGVEVHNAKTKPREEQYNSTYRVVSVLTVLHQDWLNGKEYKCKVSNKALPAPIEKTISKAKGQPREPQVYTLPPSRDELTKNQVSLTCLVKGFYPSDIAVEWESNGQPENNYKTTPPVLDSDGSFFLYSKLTVDKSRWQQGNVFSCSVMHEALHNHYTQKSLSLSPG

SEQ ID NO: 197 - protein, 281 aa, artificial sequence; identical to SEQ ID NO: 171
  TACI FC

SEQ ID NO: 198 - protein, 344 aa, ARTIFICIAL SEQUENCE
  TACI FC
SLSCRKEQGKFYDHLLRDCISCASICGQHPKQCAYFCENKLRSGGGGSGGGGSGGGGSGGGGSSLSCRKEQGKFYDHLLRDCISCASICGQHPKQCAYFCENKLRSGSGGGGSEPKSSDKTHTCPPCPAPEAEGAPSVFLFPPKPKDTLMISRTPEVTCVVVDVSHEDPEVKFNWYVDGVEVHNAKTKPREEQYNSTYRVVSVLTVLHQDWLNGKEYKCKVSNKALPAPIEKTISKAKGQPREPQVYTLPPSRDELTKNQVSLTCLVKGFYPSDIAVEWESNGQPENNYKTTPPVLDSDGSFFLYSKLTVDKSRWQQGNVFSCSVMHEALHNHYTQKSLSLSPG

SEQ ID NO: 199 - protein, 577 aa, ARTIFICIAL SEQUENCE
  TACI FC
SLSCRKEQGEYYDHLLRDCISCASICGQHPKQCADFCENKLRSGSGGGGSGGGGSEPKSSDKTHTCPPCPAPEAEGAPSVFLFPPKPKDTLMISRTPEVTCVVVDVSHEDPEVKFNWYVDGVEVHNAKTKPREEQYNSTYRVVSVLTVLHQDWLNGKEYKCKVSNKALPAPIEKTISKAKGQPREPQVYTLPPSRDELTKNQVSLTCLVKGFYPSDIAVEWESNGQPENNYKTTPPVLDSDGSFFLYSKLTVDKSRWQQGNVFSCSVMHEALHNHYTQKSLSLSPGGGGGSGGGGSGGGGSGGGGSGGGGSGGGGSGGGGSGGGGSGGGGSGGGGSGGGGSGGGGSEPKSSDKTHTCPPCPAPEAEGAPSVFLFPPKPKDTLMISRTPEVTCVVVDVSHEDPEVKFNWYVDGVEVHNAKTKPREEQYNSTYRVVSVLTVLHQDWLNGKEYKCKVSNKALPAPIEKTISKAKGQPREPQVYTLPPSRDELTKNQVSLTCLVKGFYPSDIAVEWESNGQPENNYKTTPPVLDSDGSFFLYSKLTVDKSRWQQGNVFSCSVMHEALHNHYTQKSLSLSPG

SEQ ID NO: 200 - protein, 281 aa, ARTIFICIAL SEQUENCE; identical to SEQ ID NO: 167
  TACI FC

SEQ ID NO: 201 - protein, 344 aa, ARTIFICIAL SEQUENCE
  TACI FC
SLSCRKEQGEYYDHLLRDCISCASICGQHPKQCADFCENKLRSGSGGGGSEPKSSDKTHTCPPCPAPEAEGAPSVFLFPPKPKDTLMISRTPEVTCVVVDVSHEDPEVKFNWYVDGVEVHNAKTKPREEQYNSTYRVVSVLTVLHQDWLNGKEYKCKVSNKALPAPIEKTISKAKGQPREPQVYTLPPSRDELTKNQVSLTCLVKGFYPSDIAVEWESNGQPENNYKTTPPVLDSDGSFFLYSKLTVDKSRWQQGNVFSCSVMHEALHNHYTQKSLSLSPGGGGGSGGGGSGGGGSGGGGSSLSCRKEQGEYYDHLLRDCISCASICGQHPKQCADFCENKLRS

SEQ ID NO: 202 - protein, 344 aa, ARTIFICIAL SEQUENCE
  TACI FC
SLSCRKEQGKFYDHLLRDCISCASICGQHPKQCAYFCENKLRSGSGGGGSEPKSSDKTHTCPPCPAPEAEGAPSVFLFPPKPKDTLMISRTPEVTCVVVDVSHEDPEVKFNWYVDGVEVHNAKTKPREEQYNSTYRVVSVLTVLHQDWLNGKEYKCKVSNKALPAPIEKTISKAKGQPREPQVYTLPPSRDELTKNQVSLTCLVKGFYPSDIAVEWESNGQPENNYKTTPPVLDSDGSFFLYSKLTVDKSRWQQGNVFSCSVMHEALHNHYTQKSLSLSPGGGGGSGGGGSGGGGSGGGGSSLSCRKEQGKFYDHLLRDCISCASICGQHPKQCAYFCENKLRS

SEQ ID NO: 203 - protein, 616 aa, ARTIFICIAL SEQUENCE
  TACI FC
VAMRSCPEEQYWDPLLGTCMSCKTICNHQSQRTCAAFCRSLSCRKEQGKFYDHLLRDCISCASICGQHPKQCAYFCENKLRSGSGGGGSGGGGSEPKSSDKTHTCPPCPAPEAEGAPSVFLFPPKPKDTLMISRTPEVTCVVVDVSHEDPEVKFNWYVDGVEVHNAKTKPREEQYNSTYRVVSVLTVLHQDWLNGKEYKCKVSNKALPAPIEKTISKAKGQPREPQVYTLPPSRDELTKNQVSLTCLVKGFYPSDIAVEWESNGQPENNYKTTPPVLDSDGSFFLYSKLTVDKSRWQQGNVFSCSVMHEALHNHYTQKSLSLSPGGGGGSGGGGSGGGGSGGGGSGGGGSGGGGSGGGGSGGGGSGGGGSGGGGSGGGGSGGGGSEPKSSDKTHTCPPCPAPEAEGAPSVFLFPPKPKDTLMISRTPEVTCVVVDVSHEDPEVKFNWYVDGVEVHNAKTKPREEQYNSTYRVVSVLTVLHQDWLNGKEYKCKVSNKALPAPIEKTISKAKGQPREPQVYTLPPSRDELTKNQVSLTCLVKGFYPSDIAVEWESNGQPENNYKTTPPVLDSDGSFFLYSKLTVDKSRWQQGNVFSCSVMHEALHNHYTQKSLSLSPG

SEQ ID NO: 204 - protein, 313 aa, ARTIFICIAL SEQUENCE; identical to SEQ ID NO: 132
  TACI FC

SEQ ID NO: 205 - protein, 640 aa, ARTIFICIAL SEQUENCE
  TACI FC
SRVDQEERFPQGLWTGVAMRSCPEEQYWDPLLGTCMSCKTICNHQSQRTCAAFCRSLSCRKEQGKFYDHLLRDCISCASICGQHPKQCAYFCENKLRSPVNLPPELGSGGGGSGGGGSEPKSSDKTHTCPPCPAPEAEGAPSVFLFPPKPKDTLMISRTPEVTCVVVDVSHEDPEVKFNWYVDGVEVHNAKTKPREEQYNSTYRVVSVLTVLHQDWLNGKEYKCKVSNKALPAPIEKTISKAKGQPREPQVYTLPPSRDELTKNQVSLTCLVKGFYPSDIAVEWESNGQPENNYKTTPPVLDSDGSFFLYSKLTVDKSRWQQGNVFSCSVMHEALHNHYTQKSLSLSPGGGGGSGGGGSGGGGSGGGGSGGGGSGGGGSGGGGSGGGGSGGGGSGGGGSGGGGSGGGGSEPKSSDKTHTCPPCPAPEAEGAPSVFLFPPKPKDTLMISRTPEVTCVVVDVSHEDPEVKFNWYVDGVEVHNAKTKPREEQYNSTYRVVSVLTVLHQDWLNGKEYKCKVSNKALPAPIEKTISKAKGQPREPQVYTLPPSRDELTKNQVSLTCLVKGFYPSDIAVEWESNGQPENNYKTTPPVLDSDGSFFLYSKLTVDKSRWQQGNVFSCSVMHEALHNHYTQKSLSLSPG

SEQ ID NO: 206 - protein, 333 aa, ARTIFICIAL SEQUENCE
  TACI FC
SRVDQEERFPQGLWTGVAMRSCPEEQYWDPLLGTCMSCKTICNHQSQRTCAAFCRSLSCRKEQGKFYDHLLRDCISCASICGQHPKQCAYFCENKLRSPVNLPPELDKTHTCPPCPAPEAEGAPSVFLFPPKPKDTLMISRTPEVTCVVVDVSHEDPEVKFNWYVDGVEVHNAKTKPREEQYNSTYRVVSVLTVLHQDWLNGKEYKCKVSNKALPSSIEKTISKAKGQPREPQVYTLPPSRDELTKNQVSLTCLVKGFYPSDIAVEWESNGQPENNYKTTPPVLDSDGSFFLYSKLTVDKSRWQQGNVFSCSVMHEALHNHYTQKSLSLSPGK

SEQ ID NO: 207 - DNA, 1731 bp, ARTIFICIAL SEQUENCE
  TACI FC
agtctctcttgcaggaaagagcaaggcaaattttacgaccatcttttgcgagactgtataagctgtgcgtctatttgtggacaacaccctaaacaatgtgcttatttctgtgaaaataagcttcgatctggatccggtggtggcgggtcagggggaggtggaagcgagcccaagtcctcagataagactcatacttgccccccctgtcccgcccctgaggccgaaggcgcaccgtcagtgtttttgttcccaccaaagcctaaggacacactgatgataagcagaacacctgaggtaacctgtgttgttgtggatgtaagccacgaagatccggaggttaagtttaactggtacgtggacggtgtagaagtccataatgctaagacgaagccgagggaggaacaatacaactccacgtatagagtggtctccgtcttgaccgtactccatcaagactggctcaacgggaaagagtacaagtgtaaagtctctaacaaagctcttcctgcaccgattgagaaaaccatatctaaagccaagggacaaccgagagaaccacaggtttacacgctcccccccagtagagacgaacttacaaaaaaccaggtcagtcttacctgcctcgtcaaaggcttctacccctctgacatcgctgttgagtgggaatctaacggccaacctgagaacaattacaaaacaaccccgcctgtccttgactcagacggttccttttttctttacagcaagctgaccgtcgacaaatcacggtggcaacaaggcaatgtgttttcctgttccgtgatgcacgaggcactgcacaaccactacactcaaaaatccctttccctttccccagggggaggtggagggagcggtggaggtggtagcgggggtggaggctcaggtggtgggggttccggcggtggcggaagtggaggcggtggctctggtggtggcggatctggcggaggaggcagcggcggaggtgggtctgggggtggaggctccggaggcgggggaagcggtggaggagggtcagagcccaaaagctccgacaagactcacacatgccccccttgtccagcgcctgaagctgagggtgcgccctctgtcttccttttcccccctaagccgaaagataccctgatgatctcccgcactcccgaagtcacatgtgttgttgtcgacgtatctcatgaagatcctgaggtgaaattcaactggtatgtagacggggtcgaagttcataatgctaagactaagccacgagaagagcaatacaactcaacgtatcgggtggtgagcgttctgacggttctgcaccaagattggcttaatggaaaagagtataagtgcaaggtgtccaacaaggctcttccggcacccatcgaaaagacgatttccaaagcgaaaggccaacctagggaaccgcaagtttacactttgcccccgtcaagagacgaacttaccaagaatcaagtttccctgacgtgccttgtgaagggcttctaccctagcgatatagcagttgagtgggaatctaacggccagcccgaaaataattataagactactccgcccgtgctggacagtgatggttcatttttcctgtattcaaaactcactgtggacaaatctagatggcagcagggtaatgtgttctcttgttcagttatgcacgaggcattgcacaatcactatacgcaaaaaagtttgtctctctctccgggg

SEQ ID NO: 208 - DNA, 843 bp, ARTIFICIAL SEQUENCE
  TACI FC
agtctctcttgcaggaaagagcaaggcaaattttacgaccatcttttgcgagactgtataagctgtgcgtctatttgtggacaacaccctaaacaatgtgcttatttctgtgaaaataagcttcgatctggatccggtggaggagggtcagagcccaaaagctccgacaagactcacacatgccccccttgtccagcgcctgaagctgagggtgcgccctctgtcttccttttcccccctaagccgaaagataccctgatgatctcccgcactcccgaagtcacatgtgttgttgtcgacgtatctcatgaagatcctgaggtgaaattcaactggtatgtagacggggtcgaagttcataatgctaagactaagccacgagaagagcaatacaactcaacgtatcgggtggtgagcgttctgacggttctgcaccaagattggcttaatggaaaagagtataagtgcaaggtgtccaacaaggctcttccggcacccatcgaaaagacgatttccaaagcgaaaggccaacctagggaaccgcaagtttacactttgcccccgtcaagagacgaacttaccaagaatcaagtttccctgacgtgccttgtgaagggcttctaccctagcgatatagcagttgagtgggaatctaacggccagcccgaaaataattataagactactccgcccgtgctggacagtgatggttcatttttcctgtattcaaaactcactgtggacaaatctagatggcagcagggtaatgtgttctcttgttcagttatgcacgaggcattgcacaatcactatacgcaaaaaagtttgtctctctctccgggg

SEQ ID NO: 209 - DNA, 1032 bp, ARTIFICIAL SEQUENCE
  TACI FC
agtctctcttgcaggaaagagcaaggcaaattttacgaccatcttttgcgagactgtataagctgtgcgtctatttgtggacaacaccctaaacaatgtgcttatttctgtgaaaataagcttcgatctgggggtggcggatcaggaggtggcggttcaggcggaggaggttctgggggtgggggttcttcattgtcctgcagaaaggaacaggggaaattttacgatcacttgcttagagattgtataagctgcgcgagcatttgcgggcaacaccctaaacagtgtgcgtatttctgcgagaataaactccggtctggatccggtggaggagggtcagagcccaaaagctccgacaagactcacacatgccccccttgtccagcgcctgaagctgagggtgcgccctctgtcttccttttcccccctaagccgaaagataccctgatgatctcccgcactcccgaagtcacatgtgttgttgtcgacgtatctcatgaagatcctgaggtgaaattcaactggtatgtagacggggtcgaagttcataatgctaagactaagccacgagaagagcaatacaactcaacgtatcgggtggtgagcgttctgacggttctgcaccaagattggcttaatggaaaagagtataagtgcaaggtgtccaacaaggctcttccggcacccatcgaaaagacgatttccaaagcgaaaggccaacctagggaaccgcaagtttacactttgcccccgtcaagagacgaacttaccaagaatcaagtttccctgacgtgccttgtgaagggcttctaccctagcgatatagcagttgagtgggaatctaacggccagcccgaaaataattataagactactccgcccgtgctggacagtgatggttcatttttcctgtattcaaaactcactgtggacaaatctagatggcagcagggtaatgtgttctcttgttcagttatgcacgaggcattgcacaatcactatacgcaaaaaagtttgtctctctctccgggg

SEQ ID NO: 210 - DNA, 1731 bp, ARTIFICIAL SEQUENCE
  TACI FC
agtctctcttgcaggaaagagcaaggcgaatattacgaccatcttttgcgagactgtataagctgtgcgtctatttgtggacaacaccctaaacaatgtgctgatttctgtgaaaataagcttcgatctggatccggtggtggcgggtcagggggaggtggaagcgagcccaagtcctcagataagactcatacttgccccccctgtcccgcccctgaggccgaaggcgcaccgtcagtgtttttgttcccaccaaagcctaaggacacactgatgataagcagaacacctgaggtaacctgtgttgttgtggatgtaagccacgaagatccggaggttaagtttaactggtacgtggacggtgtagaagtccataatgctaagacgaagccgagggaggaacaatacaactccacgtatagagtggtctccgtcttgaccgtactccatcaagactggctcaacgggaaagagtacaagtgtaaagtctctaacaaagctcttcctgcaccgattgagaaaaccatatctaaagccaagggacaaccgagagaaccacaggtttacacgctcccccccagtagagacgaacttacaaaaaaccaggtcagtcttacctgcctcgtcaaaggcttctacccctctgacatcgctgttgagtgggaatctaacggccaacctgagaacaattacaaaacaaccccgcctgtccttgactcagacggttccttttttctttacagcaagctgaccgtcgacaaatcacggtggcaacaaggcaatgtgttttcctgttccgtgatgcacgaggcactgcacaaccactacactcaaaaatccctttccctttccccagggggaggtggagggagcggtggaggtggtagcgggggtggaggctcaggtggtgggggttccggcggtggcggaagtggaggcggtggctctggtggtggcggatctggcggaggaggcagcggcggaggtgggtctgggggtggaggctccggaggcgggggaagcggtggaggagggtcagagcccaaaagctccgacaagactcacacatgccccccttgtccagcgcctgaagctgagggtgcgccctctgtcttccttttcccccctaagccgaaagataccctgatgatctcccgcactcccgaagtcacatgtgttgttgtcgacgtatctcatgaagatcctgaggtgaaattcaactggtatgtagacggggtcgaagttcataatgctaagactaagccacgagaagagcaatacaactcaacgtatcgggtggtgagcgttctgacggttctgcaccaagattggcttaatggaaaagagtataagtgcaaggtgtccaacaaggctcttccggcacccatcgaaaagacgatttccaaagcgaaaggccaacctagggaaccgcaagtttacactttgcccccgtcaagagacgaacttaccaagaatcaagtttccctgacgtgccttgtgaagggcttctaccctagcgatatagcagttgagtgggaatctaacggccagcccgaaaataattataagactactccgcccgtgctggacagtgatggttcatttttcctgtattcaaaactcactgtggacaaatctagatggcagcagggtaatgtgttctcttgttcagttatgcacgaggcattgcacaatcactatacgcaaaaaagtttgtctctctctccgggg

SEQ ID NO: 211 - DNA, 843 bp, ARTIFICIAL SEQUENCE
  TACI FC
agtctctcttgcaggaaagagcaaggcgaatattacgaccatcttttgcgagactgtataagctgtgcgtctatttgtggacaacaccctaaacaatgtgctgatttctgtgaaaataagcttcgatctggatccggtggaggagggtcagagcccaaaagctccgacaagactcacacatgccccccttgtccagcgcctgaagctgagggtgcgccctctgtcttccttttcccccctaagccgaaagataccctgatgatctcccgcactcccgaagtcacatgtgttgttgtcgacgtatctcatgaagatcctgaggtgaaattcaactggtatgtagacggggtcgaagttcataatgctaagactaagccacgagaagagcaatacaactcaacgtatcgggtggtgagcgttctgacggttctgcaccaagattggcttaatggaaaagagtataagtgcaaggtgtccaacaaggctcttccggcacccatcgaaaagacgatttccaaagcgaaaggccaacctagggaaccgcaagtttacactttgcccccgtcaagagacgaacttaccaagaatcaagtttccctgacgtgccttgtgaagggcttctaccctagcgatatagcagttgagtgggaatctaacggccagcccgaaaataattataagactactccgcccgtgctggacagtgatggttcatttttcctgtattcaaaactcactgtggacaaatctagatggcagcagggtaatgtgttctcttgttcagttatgcacgaggcattgcacaatcactatacgcaaaaaagtttgtctctctctccgggg

SEQ ID NO: 212 - DNA, 1032 bp, ARTIFICIAL SEQUENCE
  TACI FC
agtctctcttgcaggaaagagcaaggcgaatattacgaccatcttttgcgagactgtataagctgtgcgtctatttgtggacaacaccctaaacaatgtgctgatttctgtgaaaataagcttcgatctggatccggtggaggagggtcagagcccaaaagctccgacaagactcacacatgccccccttgtccagcgcctgaagctgagggtgcgccctctgtcttccttttcccccctaagccgaaagataccctgatgatctcccgcactcccgaagtcacatgtgttgttgtcgacgtatctcatgaagatcctgaggtgaaattcaactggtatgtagacggggtcgaagttcataatgctaagactaagccacgagaagagcaatacaactcaacgtatcgggtggtgagcgttctgacggttctgcaccaagattggcttaatggaaaagagtataagtgcaaggtgtccaacaaggctcttccggcacccatcgaaaagacgatttccaaagcgaaaggccaacctagggaaccgcaagtttacactttgcccccgtcaagagacgaacttaccaagaatcaagtttccctgacgtgccttgtgaagggcttctaccctagcgatatagcagttgagtgggaatctaacggccagcccgaaaataattataagactactccgcccgtgctggacagtgatggttcatttttcctgtattcaaaactcactgtggacaaatctagatggcagcagggtaatgtgttctcttgttcagttatgcacgaggcattgcacaatcactatacgcaaaaaagtttgtctctctctccgggggggggtggcggatcaggaggtggcggttcaggcggaggaggttctgggggtgggggttcttcattgtcctgcagaaaggaacagggggagtattacgatcacttgcttagagattgtataagctgcgcgagcatttgcgggcaacaccctaaacagtgtgcggatttctgcgagaataaactccggtct

SEQ ID NO: 213 - DNA, 1032 bp, ARTIFICIAL SEQUENCE
  TACI FC
agtctctcttgcaggaaagagcaaggcaaattttacgaccatcttttgcgagactgtataagctgtgcgtctatttgtggacaacaccctaaacaatgtgcttatttctgtgaaaataagcttcgatctggatccggtggaggagggtcagagcccaaaagctccgacaagactcacacatgccccccttgtccagcgcctgaagctgagggtgcgccctctgtcttccttttcccccctaagccgaaagataccctgatgatctcccgcactcccgaagtcacatgtgttgttgtcgacgtatctcatgaagatcctgaggtgaaattcaactggtatgtagacggggtcgaagttcataatgctaagactaagccacgagaagagcaatacaactcaacgtatcgggtggtgagcgttctgacggttctgcaccaagattggcttaatggaaaagagtataagtgcaaggtgtccaacaaggctcttccggcacccatcgaaaagacgatttccaaagcgaaaggccaacctagggaaccgcaagtttacactttgcccccgtcaagagacgaacttaccaagaatcaagtttccctgacgtgccttgtgaagggcttctaccctagcgatatagcagttgagtgggaatctaacggccagcccgaaaataattataagactactccgcccgtgctggacagtgatggttcatttttcctgtattcaaaactcactgtggacaaatctagatggcagcagggtaatgtgttctcttgttcagttatgcacgaggcattgcacaatcactatacgcaaaaaagtttgtctctctctccgggggggggtggcggatcaggaggtggcggttcaggcggaggaggttctgggggtgggggttcttcattgtcctgcagaaaggaacaggggaaattttacgatcacttgcttagagattgtataagctgcgcgagcatttgcgggcaacaccctaaacagtgtgcgtatttctgcgagaataaactccggtct

SEQ ID NO: 214 - DNA, 1848 bp, ARTIFICIAL SEQUENCE
  TACI FC
gtggcaatgcgctcatgcccagaggaacaatattgggatccgcttcttgggacgtgtatgagctgcaagaccatctgtaatcatcaatcccaaaggacatgcgcagctttctgcaggagtctctcttgcaggaaagagcaaggcaaattttacgaccatcttttgcgagactgtataagctgtgcgtctatttgtggacaacaccctaaacaatgtgcttatttctgtgaaaataagcttcgatctggatccggtggtggcgggtcagggggaggtggaagcgagcccaagtcctcagataagactcatacttgccccccctgtcccgcccctgaggccgaaggcgcaccgtcagtgtttttgttcccaccaaagcctaaggacacactgatgataagcagaacacctgaggtaacctgtgttgttgtggatgtaagccacgaagatccggaggttaagtttaactggtacgtggacggtgtagaagtccataatgctaagacgaagccgagggaggaacaatacaactccacgtatagagtggtctccgtcttgaccgtactccatcaagactggctcaacgggaaagagtacaagtgtaaagtctctaacaaagctcttcctgcaccgattgagaaaaccatatctaaagccaagggacaaccgagagaaccacaggtttacacgctcccccccagtagagacgaacttacaaaaaaccaggtcagtcttacctgcctcgtcaaaggcttctacccctctgacatcgctgttgagtgggaatctaacggccaacctgagaacaattacaaaacaaccccgcctgtccttgactcagacggttccttttttctttacagcaagctgaccgtcgacaaatcacggtggcaacaaggcaatgtgttttcctgttccgtgatgcacgaggcactgcacaaccactacactcaaaaatccctttccctttccccagggggaggtggagggagcggtggaggtggtagcgggggtggaggctcaggtggtgggggttccggcggtggcggaagtggaggcggtggctctggtggtggcggatctggcggaggaggcagcggcggaggtgggtctgggggtggaggctccggaggcgggggaagcggtggaggagggtcagagcccaaaagctccgacaagactcacacatgccccccttgtccagcgcctgaagctgagggtgcgccctctgtcttccttttcccccctaagccgaaagataccctgatgatctcccgcactcccgaagtcacatgtgttgttgtcgacgtatctcatgaagatcctgaggtgaaattcaactggtatgtagacggggtcgaagttcataatgctaagactaagccacgagaagagcaatacaactcaacgtatcgggtggtgagcgttctgacggttctgcaccaagattggcttaatggaaaagagtataagtgcaaggtgtccaacaaggctcttccggcacccatcgaaaagacgatttccaaagcgaaaggccaacctagggaaccgcaagtttacactttgcccccgtcaagagacgaacttaccaagaatcaagtttccctgacgtgccttgtgaagggcttctaccctagcgatatagcagttgagtgggaatctaacggccagcccgaaaataattataagactactccgcccgtgctggacagtgatggttcatttttcctgtattcaaaactcactgtggacaaatctagatggcagcagggtaatgtgttctcttgttcagttatgcacgaggcattgcacaatcactatacgcaaaaaagtttgtctctctctccgggg

SEQ ID NO: 215 - DNA, 939 bp, ARTIFICIAL SEQUENCE
  TACI FC
gcaatgcgctcatgcccagaggaacaatattgggatccgcttcttgggacgtgtatgagctgcaagaccatctgtaatcatcaatcccaaaggacatgcgcagctttctgcaggagtctctcttgcaggaaagagcaaggcaaattttacgaccatcttttgcgagactgtataagctgtgcgtctatttgtggacaacaccctaaacaatgtgcttatttctgtgaaaataagcttcgatctgagcccaaaagctccgacaagactcacacatgccccccttgtccagcgcctgaagctgagggtgcgccctctgtcttccttttcccccctaagccgaaagataccctgatgatctcccgcactcccgaagtcacatgtgttgttgtcgacgtatctcatgaagatcctgaggtgaaattcaactggtatgtagacggggtcgaagttcataatgctaagactaagccacgagaagagcaatacaactcaacgtatcgggtggtgagcgttctgacggttctgcaccaagattggcttaatggaaaagagtataagtgcaaggtgtccaacaaggctcttccgagctccatcgaaaagacgatttccaaagcgaaaggccaacctagggaaccgcaagtttacactttgcccccgtcaagagacgaacttaccaagaatcaagtttccctgacgtgccttgtgaagggcttctaccctagcgatatagcagttgagtgggaatctaacggccagcccgaaaataattataagactactccgcccgtgctggacagtgatggttcatttttcctgtattcaaaactcactgtggacaaatctagatggcagcagggtaatgtgttctcttgttcagttatgcacgaggcattgcacaatcactatacgcaaaaaagtttgtctctctctccggggaag

SEQ ID NO: 216 - DNA, 1920 bp, ARTIFICIAL SEQUENCE
  TACI FC
agccgtgtggaccaggaggagcgctttccacagggcctgtggacgggggtggcaatgcgctcatgcccagaggaacaatattgggatccgcttcttgggacgtgtatgagctgcaagaccatctgtaatcatcaatcccaaaggacatgcgcagctttctgcaggagtctctcttgcaggaaagagcaaggcaaattttacgaccatcttttgcgagactgtataagctgtgcgtctatttgtggacaacaccctaaacaatgtgcttatttctgtgaaaataagcttcgatctcccgtgaacctgccacccgagctgggatccggtggtggcgggtcagggggaggtggaagcgagcccaagtcctcagataagactcatacttgccccccctgtcccgcccctgaggccgaaggcgcaccgtcagtgtttttgttcccaccaaagcctaaggacacactgatgataagcagaacacctgaggtaacctgtgttgttgtggatgtaagccacgaagatccggaggttaagtttaactggtacgtggacggtgtagaagtccataatgctaagacgaagccgagggaggaacaatacaactccacgtatagagtggtctccgtcttgaccgtactccatcaagactggctcaacgggaaagagtacaagtgtaaagtctctaacaaagctcttcctgcaccgattgagaaaaccatatctaaagccaagggacaaccgagagaaccacaggtttacacgctcccccccagtagagacgaacttacaaaaaaccaggtcagtcttacctgcctcgtcaaaggcttctacccctctgacatcgctgttgagtgggaatctaacggccaacctgagaacaattacaaaacaaccccgcctgtccttgactcagacggttccttttttctttacagcaagctgaccgtcgacaaatcacggtggcaacaaggcaatgtgttttcctgttccgtgatgcacgaggcactgcacaaccactacactcaaaaatccctttccctttccccagggggaggtggagggagcggtggaggtggtagcgggggtggaggctcaggtggtgggggttccggcggtggcggaagtggaggcggtggctctggtggtggcggatctggcggaggaggcagcggcggaggtgggtctgggggtggaggctccggaggcgggggaagcggtggaggagggtcagagcccaaaagctccgacaagactcacacatgccccccttgtccagcgcctgaagctgagggtgcgccctctgtcttccttttcccccctaagccgaaagataccctgatgatctcccgcactcccgaagtcacatgtgttgttgtcgacgtatctcatgaagatcctgaggtgaaattcaactggtatgtagacggggtcgaagttcataatgctaagactaagccacgagaagagcaatacaactcaacgtatcgggtggtgagcgttctgacggttctgcaccaagattggcttaatggaaaagagtataagtgcaaggtgtccaacaaggctcttccggcacccatcgaaaagacgatttccaaagcgaaaggccaacctagggaaccgcaagtttacactttgcccccgtcaagagacgaacttaccaagaatcaagtttccctgacgtgccttgtgaagggcttctaccctagcgatatagcagttgagtgggaatctaacggccagcccgaaaataattataagactactccgcccgtgctggacagtgatggttcatttttcctgtattcaaaactcactgtggacaaatctagatggcagcagggtaatgtgttctcttgttcagttatgcacgaggcattgcacaatcactatacgcaaaaaagtttgtctctctctccgggg

SEQ ID NO: 217 - DNA, 999 bp, ARTIFICIAL SEQUENCE
  TACI FC
agccgtgtggaccaggaggagcgctttccacagggcctgtggacgggggtggcaatgcgctcatgcccagaggaacaatattgggatccgcttcttgggacgtgtatgagctgcaagaccatctgtaatcatcaatcccaaaggacatgcgcagctttctgcaggagtctctcttgcaggaaagagcaaggcaaattttacgaccatcttttgcgagactgtataagctgtgcgtctatttgtggacaacaccctaaacaatgtgcttatttctgtgaaaataagcttcgatctcccgtgaacctgccacccgagctggacaagactcacacatgccccccttgtccagcgcctgaagctgagggtgcgccctctgtcttccttttcccccctaagccgaaagataccctgatgatctcccgcactcccgaagtcacatgtgttgttgtcgacgtatctcatgaagatcctgaggtgaaattcaactggtatgtagacggggtcgaagttcataatgctaagactaagccacgagaagagcaatacaactcaacgtatcgggtggtgagcgttctgacggttctgcaccaagattggcttaatggaaaagagtataagtgcaaggtgtccaacaaggctcttccgagctccatcgaaaagacgatttccaaagcgaaaggccaacctagggaaccgcaagtttacactttgcccccgtcaagagacgaacttaccaagaatcaagtttccctgacgtgccttgtgaagggcttctaccctagcgatatagcagttgagtgggaatctaacggccagcccgaaaataattataagactactccgcccgtgctggacagtgatggttcatttttcctgtattcaaaactcactgtggacaaatctagatggcagcagggtaatgtgttctcttgttcagttatgcacgaggcattgcacaatcactatacgcaaaaaagtttgtctctctctccggggaag

SEQ ID NO: 218 - protein, 522 aa, ARTIFICIAL SEQUENCE
  FC VARIANT
EPKSSDKTHTCPPCPAPEAEGAPSVFLFPPKPKDTLMISRTPEVTCVVVDVSHEDPEVKFNWYVDGVEVHNAKTKPREEQYNSTYRVVSVLTVLHQDWLNGKEYKCKVSNKALPAPIEKTISKAKGQPREPQVYTLPPSRDELTKNQVSLTCLVKGFYPSDIAVEWESNGQPENNYKTTPPVLDSDGSFFLYSKLTVDKSRWQQGNVFSCSVMHEALHNHYTQKSLSLSPGGGGGSGGGGSGGGGSGGGGSGGGGSGGGGSGGGGSGGGGSGGGGSGGGGSGGGGSGGGGSEPKSSDKTHTCPPCPAPEAEGAPSVFLFPPKPKDTLMISRTPEVTCVVVDVSHEDPEVKFNWYVDGVEVHNAKTKPREEQYNSTYRVVSVLTVLHQDWLNGKEYKCKVSNKALPAPIEKTISKAKGQPREPQVYTLPPSRDELTKNQVSLTCLVKGFYPSDIAVEWESNGQPENNYKTTPPVLDSDGSFFLYSKLTVDKSRWQQGNVFSCSVMHEALHNHYTQKSLSLSPG

SEQ ID NO: 219 - protein, 222 aa, ARTIFICIAL SEQUENCE
  FC VARIANT
VECPPCPAPPVAGPSVFLFPPKPKDTLMISRTPEVTCVVVDVSHEDPEVQFNWYVDGVEVHNAKTKPREEQFNSTFRVVSVLTVVHQDWLNGKEYKCKVSNKGLPAPIEKTISKTKGQPREPQVYTLPPSREEMTKNQVSLTCLVKGFYPSDISVEWESNGQPENNYKTTPPMLDSDGSFFLYSKLTVDKSRWQQGNVFSCSVMHEALHNHYTQKSLSLSPG

SEQ ID NO: 220 - protein, 228 aa, ARTIFICIAL SEQUENCE
  FC VARIANT
ESKYGPPCPPCPAPEFLGGPSVFLFPPKPKDTLMISRTPEVTCVVVDVSQEDPEVQFNWYVDGVEVHNAKTKPREEQFNSTYRVVSVLTVLHQDWLNGKEYKCKVSNKGLPSSIEKTISKAKGQPREPQVYTLPPSQEEMTKNQVSLTCLVKGFYPSDIAVEWESNGQPENNYKTTPPVLDSDGSFFLYSRLTVDKSRWQEGNVFSCSVMHEALHNHYTQKSLSLSLG

SEQ ID NO: 221 - protein, 226 aa, ARTIFICIAL SEQUENCE
  FC VARIANT
DKTHTCPPCPAPEAEGAPSVFLFPPKPKDTLMISRTPEVTCVVVDVSHEDPEVKFNWYVDGVEVHNAKTKPREEQYNSTYRVVSVLTVLHQDWLNGKEYKCKVSNKALPAPIEKTISKAKGQPREPQVYTLPPSRDELTKNQVSLTCLVKGFYPSDIAVEWESNGQPENNYKTTPPVLDSDGSFFLYSKLTVDKSRWQQGNVFSCSVMHEALHNHYTQKSLSLSPG

SEQ ID NO: 222 - protein, 281 aa, ARTIFICIAL SEQUENCE
  TACI VARIANT
SLSCRKEEGKFYDHLLRDCISCASICGQHPKQCAYFCENKLRSGSGGGGSEPKSSDKTHTCPPCPAPEAEGAPSVFLFPPKPKDTLMISRTPEVTCVVVDVSHEDPEVKFNWYVDGVEVHNAKTKPREEQYNSTYRVVSVLTVLHQDWLNGKEYKCKVSNKALPAPIEKTISKAKGQPREPQVYTLPPSRDELTKNQVSLTCLVKGFYPSDIAVEWESNGQPENNYKTTPPVLDSDGSFFLYSKLTVDKSRWQQGNVFSCSVMHEALHNHYTQKSLSLSPG

SEQ ID NO: 223 - protein, 281 aa, ARTIFICIAL SEQUENCE
  TACI VARIANT
SLSCRKEEGEFYDHLLRDCISCASICGQHPKQCAYFCENKLRSGSGGGGSEPKSSDKTHTCPPCPAPEAEGAPSVFLFPPKPKDTLMISRTPEVTCVVVDVSHEDPEVKFNWYVDGVEVHNAKTKPREEQYNSTYRVVSVLTVLHQDWLNGKEYKCKVSNKALPAPIEKTISKAKGQPREPQVYTLPPSRDELTKNQVSLTCLVKGFYPSDIAVEWESNGQPENNYKTTPPVLDSDGSFFLYSKLTVDKSRWQQGNVFSCSVMHEALHNHYTQKSLSLSPG

SEQ ID NO: 224 - protein, 281 aa, ARTIFICIAL SEQUENCE
  TACI FC
SLSCRKEEGKYYDHLLRDCISCASICGQHPKQCAYFCENKLRSGSGGGGSEPKSSDKTHTCPPCPAPEAEGAPSVFLFPPKPKDTLMISRTPEVTCVVVDVSHEDPEVKFNWYVDGVEVHNAKTKPREEQYNSTYRVVSVLTVLHQDWLNGKEYKCKVSNKALPAPIEKTISKAKGQPREPQVYTLPPSRDELTKNQVSLTCLVKGFYPSDIAVEWESNGQPENNYKTTPPVLDSDGSFFLYSKLTVDKSRWQQGNVFSCSVMHEALHNHYTQKSLSLSPG

SEQ ID NO: 225 - protein, 281 aa, ARTIFICIAL SEQUENCE
  TACI FC
SLSCRKEEGKFYDHLLRDCISCASICGQHPKQCDYFCENKLRSGSGGGGSEPKSSDKTHTCPPCPAPEAEGAPSVFLFPPKPKDTLMISRTPEVTCVVVDVSHEDPEVKFNWYVDGVEVHNAKTKPREEQYNSTYRVVSVLTVLHQDWLNGKEYKCKVSNKALPAPIEKTISKAKGQPREPQVYTLPPSRDELTKNQVSLTCLVKGFYPSDIAVEWESNGQPENNYKTTPPVLDSDGSFFLYSKLTVDKSRWQQGNVFSCSVMHEALHNHYTQKSLSLSPG

SEQ ID NO: 226 - protein, 281 aa, ARTIFICIAL SEQUENCE
  TACI FC
SLSCRKEEGKFYDHLLRDCISCASICGQHPKQCADFCENKLRSGSGGGGSEPKSSDKTHTCPPCPAPEAEGAPSVFLFPPKPKDTLMISRTPEVTCVVVDVSHEDPEVKFNWYVDGVEVHNAKTKPREEQYNSTYRVVSVLTVLHQDWLNGKEYKCKVSNKALPAPIEKTISKAKGQPREPQVYTLPPSRDELTKNQVSLTCLVKGFYPSDIAVEWESNGQPENNYKTTPPVLDSDGSFFLYSKLTVDKSRWQQGNVFSCSVMHEALHNHYTQKSLSLSPG

SEQ ID NO: 227 - protein, 281 aa, ARTIFICIAL SEQUENCE
  TACI FC
SLSCRKEQGEYYDHLLQDCISCASICGQHPKQCAYFCENKLRSGSGGGGSEPKSSDKTHTCPPCPAPEAEGAPSVFLFPPKPKDTLMISRTPEVTCVVVDVSHEDPEVKFNWYVDGVEVHNAKTKPREEQYNSTYRVVSVLTVLHQDWLNGKEYKCKVSNKALPAPIEKTISKAKGQPREPQVYTLPPSRDELTKNQVSLTCLVKGFYPSDIAVEWESNGQPENNYKTTPPVLDSDGSFFLYSKLTVDKSRWQQGNVFSCSVMHEALHNHYTQKSLSLSPG

SEQ ID NO: 228 - protein, 281 aa, ARTIFICIAL SEQUENCE
  TACI FC
SLSCRKEQGKYYDHLLRDCISCASICGQHPKQCAYFCENKLRSGSGGGGSEPKSSDKTHTCPPCPAPEAEGAPSVFLFPPKPKDTLMISRTPEVTCVVVDVSHEDPEVKFNWYVDGVEVHNAKTKPREEQYNSTYRVVSVLTVLHQDWLNGKEYKCKVSNKALPAPIEKTISKAKGQPREPQVYTLPPSRDELTKNQVSLTCLVKGFYPSDIAVEWESNGQPENNYKTTPPVLDSDGSFFLYSKLTVDKSRWQQGNVFSCSVMHEALHNHYTQKSLSLSPG

SEQ ID NO: 229 - protein, 281 aa, ARTIFICIAL SEQUENCE
  TACI FC
SLSCRKEQGKYYDHLLQDCISCASICGQHPKQCAYFCENKLRSGSGGGGSEPKSSDKTHTCPPCPAPEAEGAPSVFLFPPKPKDTLMISRTPEVTCVVVDVSHEDPEVKFNWYVDGVEVHNAKTKPREEQYNSTYRVVSVLTVLHQDWLNGKEYKCKVSNKALPAPIEKTISKAKGQPREPQVYTLPPSRDELTKNQVSLTCLVKGFYPSDIAVEWESNGQPENNYKTTPPVLDSDGSFFLYSKLTVDKSRWQQGNVFSCSVMHEALHNHYTQKSLSLSPG

SEQ ID NO: 230 - protein, 281 aa, ARTIFICIAL SEQUENCE
  TACI FC
SLSCRKEQGKYYDHLLRDCISCASICGQHPKQCDYFCENKLRSGSGGGGSEPKSSDKTHTCPPCPAPEAEGAPSVFLFPPKPKDTLMISRTPEVTCVVVDVSHEDPEVKFNWYVDGVEVHNAKTKPREEQYNSTYRVVSVLTVLHQDWLNGKEYKCKVSNKALPAPIEKTISKAKGQPREPQVYTLPPSRDELTKNQVSLTCLVKGFYPSDIAVEWESNGQPENNYKTTPPVLDSDGSFFLYSKLTVDKSRWQQGNVFSCSVMHEALHNHYTQKSLSLSPG

SEQ ID NO: 231 - protein, 281 aa, ARTIFICIAL SEQUENCE
  TACI FC
SLSCRKEQGKYYDHLLRDCISCASICGQHPKQCADFCENKLRSGSGGGGSEPKSSDKTHTCPPCPAPEAEGAPSVFLFPPKPKDTLMISRTPEVTCVVVDVSHEDPEVKFNWYVDGVEVHNAKTKPREEQYNSTYRVVSVLTVLHQDWLNGKEYKCKVSNKALPAPIEKTISKAKGQPREPQVYTLPPSRDELTKNQVSLTCLVKGFYPSDIAVEWESNGQPENNYKTTPPVLDSDGSFFLYSKLTVDKSRWQQGNVFSCSVMHEALHNHYTQKSLSLSPG

SEQ ID NO: 232 - protein, 281 aa, ARTIFICIAL SEQUENCE
  TACI FC
SLSCRKEQGKFYDHLLQDCISCASICGQHPKQCDYFCENKLRSGSGGGGSEPKSSDKTHTCPPCPAPEAEGAPSVFLFPPKPKDTLMISRTPEVTCVVVDVSHEDPEVKFNWYVDGVEVHNAKTKPREEQYNSTYRVVSVLTVLHQDWLNGKEYKCKVSNKALPAPIEKTISKAKGQPREPQVYTLPPSRDELTKNQVSLTCLVKGFYPSDIAVEWESNGQPENNYKTTPPVLDSDGSFFLYSKLTVDKSRWQQGNVFSCSVMHEALHNHYTQKSLSLSPG

SEQ ID NO: 233 - protein, 281 aa, ARTIFICIAL SEQUENCE
  TACI FC
SLSCRKEQGKFYDHLLQDCISCASICGQHPKQCADFCENKLRSGSGGGGSEPKSSDKTHTCPPCPAPEAEGAPSVFLFPPKPKDTLMISRTPEVTCVVVDVSHEDPEVKFNWYVDGVEVHNAKTKPREEQYNSTYRVVSVLTVLHQDWLNGKEYKCKVSNKALPAPIEKTISKAKGQPREPQVYTLPPSRDELTKNQVSLTCLVKGFYPSDIAVEWESNGQPENNYKTTPPVLDSDGSFFLYSKLTVDKSRWQQGNVFSCSVMHEALHNHYTQKSLSLSPG

SEQ ID NO: 234 - protein, 281 aa, ARTIFICIAL SEQUENCE
  TACI FC
SLSCRKEQGKFYDHLLRDCISCASICGQHPKQCDDFCENKLRSGSGGGGSEPKSSDKTHTCPPCPAPEAEGAPSVFLFPPKPKDTLMISRTPEVTCVVVDVSHEDPEVKFNWYVDGVEVHNAKTKPREEQYNSTYRVVSVLTVLHQDWLNGKEYKCKVSNKALPAPIEKTISKAKGQPREPQVYTLPPSRDELTKNQVSLTCLVKGFYPSDIAVEWESNGQPENNYKTTPPVLDSDGSFFLYSKLTVDKSRWQQGNVFSCSVMHEALHNHYTQKSLSLSPG

SEQ ID NO: 235 - protein, 281 aa, ARTIFICIAL SEQUENCE
  TACI FC
SLSCRKEQGKFYDHLLRDCISCASICGQHPKQCADFCENKLRSGSGGGGSEPKSSDKTHTCPPCPAPEAEGAPSVFLFPPKPKDTLMISRTPEVTCVVVDVSHEDPEVKFNWYVDGVEVHNAKTKPREEQYNSTYRVVSVLTVLHQDWLNGKEYKCKVSNKALPAPIEKTISKAKGQPREPQVYTLPPSRDELTKNQVSLTCLVKGFYPSDIAVEWESNGQPENNYKTTPPVLDSDGSFFLYSKLTVDKSRWQQGNVFSCSVMHEALHNHYTQKSLSLSPG

SEQ ID NO: 236 - protein, 281 aa, ARTIFICIAL SEQUENCE
  TACI FC
SLSCRKEQGEYYDHLLRDCISCASICGQHPKQCAYFCENKLRSGSGGGGSEPKSSDKTHTCPPCPAPEAEGAPSVFLFPPKPKDTLMISRTPEVTCVVVDVSHEDPEVKFNWYVDGVEVHNAKTKPREEQYNSTYRVVSVLTVLHQDWLNGKEYKCKVSNKALPAPIEKTISKAKGQPREPQVYTLPPSRDELTKNQVSLTCLVKGFYPSDIAVEWESNGQPENNYKTTPPVLDSDGSFFLYSKLTVDKSRWQQGNVFSCSVMHEALHNHYTQKSLSLSPG

SEQ ID NO: 237 - protein, 281 aa, ARTIFICIAL SEQUENCE
  TACI FC
SLSCRKEQGEFYDHLLRDCISCASICGQHPKQCADFCENKLRSGSGGGGSEPKSSDKTHTCPPCPAPEAEGAPSVFLFPPKPKDTLMISRTPEVTCVVVDVSHEDPEVKFNWYVDGVEVHNAKTKPREEQYNSTYRVVSVLTVLHQDWLNGKEYKCKVSNKALPAPIEKTISKAKGQPREPQVYTLPPSRDELTKNQVSLTCLVKGFYPSDIAVEWESNGQPENNYKTTPPVLDSDGSFFLYSKLTVDKSRWQQGNVFSCSVMHEALHNHYTQKSLSLSPG

SEQ ID NO: 238 - protein, 5 aa, ARTIFICIAL SEQUENCE
  Hinge
EPKSS

SEQ ID NO: 239 - protein, 5 aa, artificial sequence
  hinge
EPKSC